European Patent Specification EP 3 331 355 B1, published April 3, 2024. Title: PATHOGEN-RESISTANT ANIMALS HAVING MODIFIED CD163 GENES. Applicant: Curators of the University of Missouri Prather, Randall Wells, Kevin Whitworth, Kristin. The sequence listing filed with the application follows.

SEQUENCE LISTING (121 sequences)

SEQ ID NO: 1 - DNA, 23 bp, Sus scrofa
ggaaacccaggctggttggaggg

SEQ ID NO: 2 - DNA, 23 bp, Sus scrofa
ggaactacagtgcggcactgtgg

SEQ ID NO: 3 - DNA, 23 bp, Sus scrofa
cagtagcaccccgccctgacggg

SEQ ID NO: 4 - DNA, 23 bp, Sus scrofa
tgtagccacagcagggacgtcgg

SEQ ID NO: 5 - DNA, 23 bp, Sus scrofa
ccagcctcgcccagcgacatggg

SEQ ID NO: 6 - DNA, 23 bp, Sus scrofa
ctttcatttatctgaactcaggg

SEQ ID NO: 7 - DNA, 23 bp, Sus scrofa
ttatctgaactcagggtccccgg

SEQ ID NO: 8 - DNA, 23 bp, Sus scrofa
cagctgcagcatatatttaaggg

SEQ ID NO: 9 - DNA, 23 bp, Artificial sequence
  Synthetic oligonucleotide
ctcctcgcccttgctcaccatgg

SEQ ID NO: 10 - DNA, 23 bp, Artificial sequence
  Synthetic oligonucleotide
gaccaggatgggcaccaccccgg

SEQ ID NO: 11 - DNA, 23 bp, Artificial sequence
  Synthetic oligonucleotide
ctctccctcactctaacctactt

SEQ ID NO: 12 - DNA, 22 bp, Artificial sequence
  Synthetic oligonucleotide
tatttctctcacatggccagtc

SEQ ID NO: 13 - DNA, 23 bp, Artificial sequence
  Synthetic oligonucleotide
ctctccctcactctaacctactt

SEQ ID NO: 14 - DNA, 22 bp, Artificial sequence
  Synthetic oligonucleotide
gactggccatgtgagagaaata

SEQ ID NO: 15 - DNA, 27767 bp, Sus scrofa
atacaagtgccttttacagacaatctgcacaagttatttgttagacatatttgattatagaattaatattaaaaggggttataacaatcaagcattgataatttaattatgtttgcctattttactttagttttttgacataactgtgtaactattgcgatttttttattcctaatgtaattagttcaaaacaaagtgcagaaatttaaaatattcaattcaacaacagtatataagtcaatattccccccttaaatttttacaaatctttagggagtgtttctcaatttctcaatttctttggttgtttcatgtcccatatggaagaaaacatgggtgtgaaagggaagcttactcttttgattacttcccttttctggttgactccacctccattatgaagcctttctgtatttttgtggaagtgaaatgatttttagaattcttagtggttctcttcttcaggagaacatttctaggtaataatacaagaagatttaaatggcataaaaccttggaatggacaaactcagaatggtgctacatgaaaactctggatctgcaggtaaaatcttctcatttattctatatttaccttttaaatagagtgtagcaatattccgacagtcaatcaatctgatttaatagtgattggcatctggagaagaagtaacagggaaaaaggcaataagctttataaggggaacttttatcttccatagactcaaaattgaagacgtgactagaagattgctagatttggcatcagttttgtaaaattgctgaggtgaaattaagtaagggatgaaaattaactaaattgtgttgagtatgaaactagtagttgttagaaaagatagaacatgaaggaatgaatattgattgaaagttgatgacctagaggacatttagactaacacctctgagtgtcaaagtctaatttatgatttacatcgatgcgttaaactcatttaacattcttacttttttcccctcaagcatttaagctgaagtataacatttcacatgaaagcctggattataaatgcacagttcagtgacctatctcagaggagtgactgccatagcattttttttgtctttttgccttcagagccacagcaacgcgggatccgaagccgcgtctgcgacccacaccacagctcacggcaatgccggatctttaacccactgagcgaggccggggatcgaacccgcagtctcatggttcctagtaggattcgttaaccactgcgccacgacgggaactcctaccatagcatttttacttttaagttactgttggtttagagtaagaaggagaaatgagagtgatggagcgtttgctatatttggagacaaggtcctatattggaggttctcaaatataaattttgtcgctttttcctccaatgtattgttcaactactatttagcaggccactgtgccaggtactggtgaaactggtgaacatgatagatgtaattcattccctcatggaactttccatctaacaatgtggatcaggtaggcttggagatgagaatgccagtggttgactatgactctgtggctgaagggagagctactcacttcgtagtttcatcaatgtctttttggttttccaggttttaagccctgctcttgcaattcttttcccttctccaactttcttctaatttctcacccctaggatgcctataaacatgagtattttcaaagctacttcactgaggttatatgatcctggtgtgaatttttcctgcctgacttgccatttagaaggaagtgtttcctggaatttccattgtggcttggtggttaaagaccctgcattgtctctgtgaggatgtgggttcaatctctggcctcattcagtgagtgggttaaggatctggtgtcgctgcaagctgtggctaagatcccacattgccatgtctgtggtgtagactggcacctggagctctgatttgaccacaatcttaggaacttcagatgtggccataaaaaggaaaaaaaagttaggaagggttttctgtcttgtttggaccttcgttaatctcaaacctttggaaccatctctcctccaaaacctcctttgggtaagactgtatgtttgccctctctcttcttttcgcagactttagaagatgttctgcccatttaagttccttcactttggctgtagtcgctgttctcagtgcctgcttggtcactagttctcttggtgagtactttgacaaatttacttgtaaccgagcccaactgtgacaagaaacactgaaaagcaaataattgctcctgaagtctagatagcatctaaaaacatgcttcatggtttcaaggatcatatattgaaaccccagggatcctctagagtcgacctgcagcatgcaggggggggggggggggggggggggggggggggggggggggggggggggggggggggggggggggggggggggggggggggggggggggggggggggggggggggtgcataaggaaagactatctcaacgtcttattcctcagcttacattagatttgaaactctagtcacctaaaatgcaaatctcatttacttaccatcagagatattaatgacctatagaattcagcataaataaagtttcatgtatggatattagcttatggttctagtcactgctaattgaaacctgtgatattgctgtttgttttgactcctatgaaataacattctcccattgtaccatggatgggtccagaaacatttctcaaatcctggcttgaaaaaataaataagtaatctaaagaataataattctctacttgctctttgaatcttgaccaattgctgcatttacctattgttacaggaggaaaagacaaggagctgaggctaacgggtggtgaaaacaagtgctctggaagagtggaggtgaaagtgcaggaggagtggggaactgtgtgtaataatggctgggacatggatgtggtctctgttgtttgtaggcagctgggatgtccaactgctatcaaagccactggatgggctaattttagtgcaggttctggacgcatttggatggatcatgtttcttgtcgagggaatgagtcagctctctgggactgcaaacatgatggatggggaaagcataactgtactcaccaacaggatgctggagtaacctgctcaggtaagacatacacaaataagtcaagcctatacatgaaatgctttgtgggaaaaaatgtatagatgagttaaaaacaaaaaggaaccagttttctataagtcatctagtccatgtataaaattacccaatccattactaaaagaccacttctggtattttacacatgacaaagcccatattaaaaaaaaaaaattcagaagagattctgaatgctataataaatgagcaagtgactagcttcaattttatattaggtcattctaccttctacttctacatgaaaatatcataatgtctaagttaattccttgtcccctttcccaataaagcactgctttcatgcactggcctatgaatcatgaactttttgccctttaactgatgatcaacttaccaaatcaagaaataaatattcttagcactgatccttttttgttgttgttggaggaagaatgttttgcaaagtagaattgcttttttctgtttaacagtgctattcatttcatttacatggtcgttttaatttataaaacatttcataagtttcacctcatatgcccttacaataactcaggaagttatatgttagacctttctgctgacaaatcccagagtcatgtttctgacccagttcagattccttggcttcccatttctctttgctcatgtcattgacctttatgcagccctcttacctcccacctttctattacagaccatctcctccataggactggtgttagaaagtactaatctctacccaggcattgtggtgcaatgtgggcagcacaggctggtatctagaaaaatgctgaagtgaattccagctcagctgctcgttaatactatcgttttaagtaagctgttcaatcctttgaaattcactttctgagcactcagtgatataataaatgtagagctactggtacactgtctggtatgtaataggtgttaccaattaaccttagtttcctcatgggtcactggttctcattacctagacaactcatttctctttcttcctctttctctttctccattctcctcctccttcttcctcttcttcttgtctgttattgttatatcattttgctgagaaagttaagaaataacaactctaacctctacatcgaccacctagagcaaagttaaaaataataataaaccttgccagactcttactataattgttgctgtctatagagttgactgtttaagttaagacatcagtatatatttttaatttttgtgttttttttttcatacttttacatgaggatcctttatataaggatgagttaaacaaacttgatttttgaagtttatacccctgaggctcaactgcataataatagaaagggatccatagcctctcaaggacttaactagtttcatgagttttcagaatctgaatttctgagattctccaccccaattaaagctcaagcctcagaacatatatccttctcttggtaaattctattcttatcacatgcgtaataataaaaaagagagatgttggagacagatttttttcctcacattctgtctctactgttttctaggtgtttgattctgtgttatttaacctcagtttgcttatctgtgaagtagggattatggtaataacatataatgctttatgttgtaaagactaaagaagatagcatatgtaacacatttggaacagggaatgcatattttgattgtgagctcttattattattaccattcagccctaataaaaatcttggtaagtggaaggctttggatttcagaacttttaaaatctaattactttttcaaaaaagaacttcttagggttttttttttttaaccacaaagtgtttctattttttaggtgtcccaaaatttcgttccaaatatctttttctcagatattttagtcctcatagaacacctagggatagtggatagagaaaattttctttattaaaaagctgttctttgctaaaaattgtagcaggtacttttgggaggggggaaaactttgattcagaaactgctaagacatggagtgttttgactaatttttcctcaatttttaatgttttttataccatagggtacttttgcaaactattatgcatacttatatatttttacttttttcctgtcttttaacttccaaattcaacttcagacaattattcatgcactaaactgtttgtagtaagaaagattaaaattaaaaaattaaccattcaacaaatgactggtttgccatttttactactttgttgtatgaacaatttttttttctacaaatgaatactttgagtctgatttatccattcctacataaaagtttttactatatcttagtattggaaggaaacaaaacaaaacacaatgtaaattttaatctataaattttgggggggtaaatatacatagatgaaagtcttaaccattaattagagtcaaaagattaaaattctccaatatgtgaacttaggctgcatccaaaatgaagcatcatttttaaggacagcatcaaaagtgaccagaggaattttactttctttcttttttttttttttgaattttagtttctaaactcacttctgaataaatacaacttctaaattctcgtcttttctctactctagatggatctgatttagagatgaggctggtgaatggaggaaaccggtgcttaggaagaatagaagtcaaatttcaaggaacgtggggaacagtgtgtgatgatcacttcaacataaatcatgcttctgtggtttgtaaacaacttgaatgtggaagtgctgtcagtttctctggttcagctaattttggagaaggttctggaccaatctggtttgatgatcttgtatgcaatggaaatgagtcagctctctggaactgcaaacatgaaggatggggaaagcacaattgcgatcatgctgaggatgctggagtgatttgcttaagtaaggactgacctgggtttgttctgttctccatgagagggcaaaaaaaggggagtaaaagtcttaaaagctcaaactgttaaaaacataatgatgattgcttcttttatcatcttattattatctaatttcaggtcgaaattctagtacctgtgcagttttttaccttaactgaaattaagataaataggatagggaggaaggatgagcagtgacatttaggtccaagtcatgaggttagaaggaaatgttcagagaatagcccattccctcagccctcaaagaaagaaagaaagaaaaagaaaaaaaaaaagaaagcttaactagaaaattttgttctctggatgttttagaggcaaaccatccctttatcattcctacctacaaagccttctcttaatcacattacccaccctttcctactatagtcaggggggggggggggggggggggggggggggggggggggggggggggggggggggggggggggggggggggggggggggggggggggggggggggggggggtgaaaaaagaaccaaacaatttcaacaaaaaaccaaacaattccaacaaaattggtccaataagcaaacctctagataaatttcagtgccctggatgttttgttaggaactcttcctacaatgcgtgctttccattctgaaaagtcctatctacttgcctgatccacttctccttccatcctaaacgattttcagtggtagtatattactgttgtctctgtctctacttatatatcttccccttttcactcactcctctcaggtacagctcttcagtttgcccttattcttgtttccttgtcaatgacttgttttgtgtccctcttacagatggagcagacctgaaactgagagtggtagatggagtcactgaatgttcaggaagattggaagtgaaattccaaggagaatggggaacaatctgtgatgatggctgggatagtgatgatgccgctgtggcatgtaagcaactgggaggtccaactgctgtcactgccattgtcgagttaacgccagtgagggactggacacattggctcacacacatacagccatgacacgatctgctctatggtccgatgattaaaggggggggggggggggggggggggggggggggggggggggggggggggggggggggggggggggggggggggggggggggggggggggggggggggggggagaagagctggtggacatttctggaaaggaaccaaaacccggaagggccttgttcttcaggatttgggatggattggggagggagaaaattgtttctaatatttcttggtgggaattcttttacagttgtgacaaatctttcacatattcttcatttgagtagtttggagggttgtctgactgttttctataataaatgtcccaagtgctatgaggtaccacatttcaaattctaattctacctgaagctccaaaaagacaaaatgttataggtcttttctttatatctaatttgcttatggtttttagccattgacaatttttttttcttaactcttgaaactataaccctatttctaaccaaattcatgttctatactggctcttcaaaaacccaggagatgggaaagccagaatctccagtgtttcagcttctgggaaggagcaagtttttaaaaataccctctgggagctaaattccacatgtatctatggcctaagtgtatgtttattttgcagatggatcagatctggaactgagacttaaaggtggaggcagccactgtgctgggacagtggaggtggaaattcagaaactggtaggaaaagtgtgtgatagaagctggggactgaaagaagctgatgtggtttgcaggcagctgggatgtggatctgcactcaaaacatcatatcaagtttattccaaaaccaaggcaacaaacacatggctgtttgtaagcagctgtaatggaaatgaaacttctctttgggactgcaagaattggcagtggggtggacttagttgtgatcactatgacgaagccaaaattacctgctcaggtaagaatttcaatcaatgtgttaggaaattgcattctactttcttttacatgtagctgtccagttttcccagcaccacttgttgaagagactgtcttttcttcatcatatagtcctacatcctttgtcataaattaattgaccataggtgtgtgggtttatatctgggctctctattctgttcctttgatctatatgtctgtttttatgccagcaccatgctgttttgattactatagctttgtagtatcatctgaagtcaggaaacatgattcctccagctttgttcttctttctcaagattgttttgtctattcagagtttatgttcccatgcagatttaatttttaaatttatttaatttttattttttatttttaatttaaattaatttaaattttttatttcccaacgtacagccaagggggccagggtaacctttacatgtatacattaaaaatttcaggtttttcccccacccatttctttctgttggcaagtaaatttttgaacaaagtttcccaatgctttttaaggggaattcccttggggggggggggggggggggggggggggggggggggggggggggggggggggggggggggggggggggggggggggggggggggggggggggggggggggggggggggggggggagacgaaattgactatattttctttgttgggaatcttttacagttgtgacaaatctttcacatattcttcatttgagtagtttggagggttgtctgactgttttctataataaatgtcccaagtgctatgaggtaccacatttcaaattctaattctacctgaagctccaaaaagacaaaatgttataggtcttttctttatatctaatttgcttatggtttttagccattgacaatttttttttcttaactcttgaaactataaccctatttctaaccaaattcatgttctatactggctcttcaaaaacccaggagatgggaaagccagaatctccagtgtttcagcttctgggaaggagcaagtttttaaaaataccctctgggagctaaattccacatgtatctatggcctaagtgtatgtttattttgcagatggatcagatctggaactgagacttaaaggtggaggcagccactgtgctgggacagtggaggtggaaattcagaaactggtaggaaaagtgtgtgatagaagctggggactgaaagaagctgatgtggtttgcaggcagctgggatgtggatctgcactcaaaacatcatatcaagtttattccaaaaccaaggcaacaaacacatggctgtttgtaagcagctgtaatggaaatgaaacttctctttgggactgcaagaattggcagtggggtggacttagttgtgatcactatgacgaaaccaaaattacctgctcaggtaagaatttcaatcaatgtgttaggaaaattgcattctactttcttttacatgtagctgtccagttttcccagcaccacttgttgaaaaaactgtctttttcttcatcatatagtcctacatcccttggccataaattaattgaccataaggggtgtgggtttaatatccggggctcctcaattcgggtcccttggatcctaaaagccggttttataacccgacacatggcctgtttttgactaaataaaacctttggaaaacaatcccgaaggtcgaggaacatggaatccccccaacaaaggaccttctttccccaaaaatgcggctcagccaactcaaaaagattttatgaatcacaaaccgcacattatcttcctaaaattactattcctatgttttaatttgcaaagtcattccgatatagttggcgcagagtaactcatttagatatccaccccaccagttcctcactcaagtaaggggggggggggggggggggggggggggggggggggggggggggggggggggggggggggggggggggggggggggggggggggggggggggggggggggcccccatgtgagattttgtgtgtcctttaagagtggagtctctatttcccactgctctctggttctccccaaagtaagccctgctggctttcaaaacttctgggagcttgccttcttggtataggactcctgggctagggagtctaatgtttggcttagaccccttactgcttgggaagaatctctgcaactgtaatgaattatcttcctatttgtgggttgctgaggatatggtcttaactgttctgtgttctacccctcctatccatcttgttgtggttccttctttatatctttagttgtagaaaagtttttcttatcaacagttgctctgtaaattgtaacttgggtgtacacctagtaggaggtgagctcagggtcttcctactctgccatcttggccatgtcctctaaacattttggtgtatttcactgcaacctttttaaaaatctcaaaagtgagctgtgattggctagtcttgtggataatctctagcatttgatgctaatcatatttatacaaatactttgttgaaaagtgatgcctttttaactattattaaaaaacgtattgacataactattgctattatactgaaaagaaagaccttagagaaaatagcataagagcaaaaccattaaacatggagacatctagtcatagggtggaaattttatgtggtccatatcccctaaccagtggctttacaccaggcacatcctaactaagatctgctcccaagtgtcttccctgatgctttaaattgtgttacatggaaactatcctttgatgaagaaatgcaaccttttaaaatacaacattgaaacttttgtgctttaattttgcttttcaacattttttctttttaaaagaagaaatttatttgtttttttaaattttaatggccacggcatatggaagttctcaggccagggatagaattcaagccacaggtgcgacccatgccacaactgctgcaacaccagatcctttaacccactgcaccaggccagggattgaagccttgccttactgacaatctgagccacttcagtcagataaagaaatttcttcattaagcagagtattcacatggtttaaacttcaaaatattaaagtgtaaactctttccccaccactgtccccagctcaccaactctacttaccacagacaactgatgtggttagggtatttaaatagtaaatccaagaaaatataaacaaatccgtatatataggtttcaccccattttattatcctaatgttgcatatcatataaactatactgtcccttgggtattcacttagtaaaatattttgatcataatttcctatcagtatttaaagagctttctgaaattatttctgtataacatttcttttctcatcggtaggggggggggggggggggggggggggggggggggggggggggggggggggggggggggggggggggggggggggggggggggggggggggggggggggggaatgggaagaaaaaaccaccatggttaattttttttatccctctacacccgggaaaattacccttggggccacacttttctatagaaaggggattatttaaaagggtctgaaaaagaatttttttttcgaaaggggaaatatttggcctaacttagtcacataagccatgttctctggcaagttaggtaacatacatttttgtcattgggggcaacaaaaacaattttccttttggaccttttgggactccgcattggttagggaaggggaagtatattggaattcggaaaattccttccaaattaaaaaaggtttgttattttcatattaacctatttcatattaattagcatgaattccagcgccattaaaagggaaaacacctggagtggtaagaaaaaagtttttttttctctttttttttttttttttttaatggccacatctgtggcatgtgaagttcccaggctaggggtcgaataggagctacagctgccagcttgcaccacagccacaacaatgccagagccaagcctcatctgcgacctataccacaactcatggcaatgctggttccttaaccccctgagtgaggcctggggtcaaacccacatcctcatggatactaaccggctttgttaccgctgagccatgagggaaactccctttttctcattgaaaataagtcaaatagataagcagcttaaggctgtttgggtgattctgtggtccagtaattatcaaatcctactggacaagaatagagaatgtgcaaatgagggaacgtgttggtgagatcaggctctgcccactgagctatcctctgtcatgggccctgtgctgttctcagagctgtacttcctagggcattgttctcatttcaattctgagttcagtgtggagagtatacgtgtgtgggggctgcacgcttttcacaacccactttctgctgatactgatttagggatccttggattgctttacagttgagtcatcattaactagtgtcacttgccttcaaagtcagcaaaataattgtctccaaactagtaggcttctagtgtatttgctttaatccaatgccatgtgaaagtaacatggtcaaagaataagttatataccttgacctaccctgtgaccaggctcttcctcttaatttattgaccactgccttaaggtcatttgaaaccatgggtttgggaggaaggcaaggcctaaatcccgtctttgttggaaggctcactgtccttgtctttagagcatcatttttttttaaactggggtacagtttatttacagtgttgtgtcaatttctgctgtacagcacagtgacccagtcatacacatacatacattctttttctcatactatcttcaattttattttctgctaagtctgccattttatcatcacctcagtttgaaggacaggatatttagagtttgttttttttttccccccaatcctgcaatttctaaattataagactctcaattagccgtatataacagctgcaggcacaggatgtctccctcacaaaattggtatttttccttccatttcttcttgcagtttggctatttcttgtctgagttcatctctctttttaagtgttaaaaagggcaaggaggattcatgctatgtcaacattatgattttttcttttctatacttgataagagtatacttttcccaaatgtcatccaacttttcagcatcagtttggacatggttttcttttcaaggtggtatttctctaatgtcacttgaataacaagactcgttagttctccaggctacaatatcctagtctgagtatattctgcatgttaattctattcagccacatccataatttaggttttattcctggaacacctcacttttttttttttttttggtctttttatagccataaccatggcatatggaggttcccaggctaggggtctaatctgagctttagccactggcccatgccacagccacagccatgccacatctgagccacatctgtgaccttttccacagctcacagaaacaccagatccctaacccactgagtgaggccaggggtcaaacctgtaacccttccatggttcctagtcagattcgttcctctgtaccacgatgggaattcctaatacctcacttatgataacacattctgaattatttaggattctattatactgcatgtaatagaaatcccaaatagcaaaatttgcaacttaaggcaggttcctgtctttacaaaatcatgttttcctttgctatatgtgcactttgctttcctctgtgaattcccttttttgttatatttctatagcttttggaaacacttttacttatttgggggggcctagatttttaaccctctccttgtttttctagaaatagagtttataattttatttcttcatttacttgatactttcaagagattcccaggaaaaaaattatggaaatactgtctctgtgcctgccaagttcaaactaagaattgtataatctgttttaattcttaagcatttatagatgacaaggctttgtgtctgataggggccagcgaactcagtaaagagggaagatgagaaagataatggcaagaatttatccctgaagtgtagttttgacaaaccagtcacaaagaggtctaagaaattttggtcacaaagttgttttgaatcccaggcattttatttgcaatgattgcatatgttctggaaaggacatctgaacctaagaaatagttcatttgcattgtgttatattttactaaggtctgagaaataatcttgagatgagaatgaactctacttcttcagagtctggaaggaataaattatgaaaatgtattaatgcttctttaaaccatattgtatatttatctattactaaacaaaaagaagtagctctatttatttatttatttatttatttatttatgtcttttgtctctttagggccacacctgtggcatatggaggttcccaggctagaggtccaattggagatgtagcagccagcctatgccagagccaccgcaacacgggatctgagccacgtctgtgacttacaccacagctcacagcaacgcctgatcctcaacccactgagcgaggccagggatcgaacccatgtcctcatggatgctagttgggttcgttaactgctgagccatgatgggaactccaaattaattatttcttatatttgttcttcatatattcatttctatagaaagaaataaatacagattcagttaatgatggcaggtaaaagcttaacttattaatcaaaggagttaatccaggcacaaaaattcaattcatggctctctgttaaaatttaggtataggtttagcaggaagaaaaggttagtagatgcagactattacatttagaatggatggacaatgaagtcctactatacagcacagggaactatatccaatctcttgggatagaatatgatggaagacaaaatcagaacaagagagtatatatatatgtgtgtgtgtgtgtgtgtgtgtgtgtgtgtgtgtgtgtgtgtgtgactgggtcaccctgcggcacagcagaaattggcagaacattgtaaatcaactatactttaataggaaaaatacttttaagggctaaatttccaatattctaaccatgtacacagagtaaatgtcataaggatgccagtctgtgtagagattgatgtgttactagcagattcatgaaataaaggctgaggatgtagtccccaagtcacttctgagtggaagaatttctcctttgtcctggactcaaatattttaggataaaggaaaaaagaagatatttatagaagggacttgttttcaagtacttgacaaaatttcaccattaaagagaaatttgtgggagttcccatcgtggctcagtggaaacaaatccaactaggaaccatgaggttgtgggtttgatccctggcctcactcagtgggttaaggatccggtgttgccgtgagctgtggtgtaggttgcagacacggttctgatcctgcgttgctgtggctgtggctgtggtgtaggccagcagcaaacagctctgattagacccctagcctggaaacctccatatgccacaggtgcagccctaaaaagacaaaaaaagagaaaagacaaaaaaaaaaaaaaaaaaaaaaaaaaaaaaaaaaaaaaaaaaaagaacccccagaggtatttatttgtttttgccttttttcactgactgttctttgtttgtttgtttgagactgatctagaagactagagattacaagaaatatggatttggctcactctaagaaactgctttcattccaaggtttgggtctatccaaaagtggaatagaatcatatgaatactagtttatgagtatttagtgagaggaatttcaagctcaaataatgattcagcaagattaaattaaggagggaattttccttgtggctgagtgggttaaggacccaatgttgtctctgtgaggatgtaggttccatcctgggctttgctcattaggttaaggatctggcattgctgcagctcagacccagtgctgccctggttgtggcttaggccaaagctgcagctccaattcaatctctggcctgggaacctccatgtgctacaaggtgcggccttaaaaggaaaaaaaaaaaattaaatcaaggactcaagagtctttcattatttgtgttgtggaagctatatttgttttaaagtcttagttgtgtttagaaagcaagatgttcttcaactcaaatttgggagggaacttgtttcatacatttttaatggataagtggcaaaattttcatgctgaggtgatctatagtgttgtaatgcagaatatagtcagatcttgaacattttaggaagttggtgagggccaattgtgtatctgtgccatgctgataagaatgtcaagggatcacaagaattcgtgttatttgacagcagtcatctttaaaaggcatttgagaaagtccaatttcaaatgcatttcctttctttaaaagataaattgaagaaaataagtctttatttcccaagtaaattgaattgcctctcagtctgttaaaagaaactcttaccttgatgattgcgctcttaacctggcaaagattgtctttaaaatctgagctccatgtcttctgctttatttctggtgtgcctttgactccagattacagtaaatggaggactgagtatagggctaaaaagtagagagaatggatgcatattatctgtggtctccaatgtgatgaatgaagtaggcaaatactcaaaggaaagagaaagcatgctccaagaattatgggttccagaaggcaaagtcccagaattgtctccagggaaggacagggaggtctagaatcggctaagcccactgtaggcagaaaaaccaagaggcatgaatggcttccctttctcacttttcactctctggcttactcctatcatgaaggaaaatattggaatcatattctccctcaccgaaatgctatttttcagcccacaggaaacccaggctggttggaggggacattccctgctctggtcgtgttgaagtacaacatggagacacgtggggcaccgtctgtgattctgacttctctctggaggcggccagcgtgctgtgcagggaactacagtgcggcactgtggtttccctcctggggggagctcactttggagaaggaagtggacagatctgggctgaagaattccagtgtgaggggcacgagtcccacctttcactctgcccagtagcaccccgccctgacgggacatgtagccacagcagggacgtcggcgtagtctgctcaagtgagacccagggaatgtgttcactttgttcccatgccatgaagagggtagggttaggtagtcacagacatctttttaaagccctgtctccttccaggatacacacaaatccgcttggtgaatggcaagaccccatgtgaaggaagagtggagctcaacattcttgggtcctgggggtccctctgcaactctcactgggacatggaagatgcccatgttttatgccagcagcttaaatgtggagttgccctttctatcccgggaggagcaccttttgggaaaggaagtgagcaggtctggaggcacatgtttcactgcactgggactgagaagcacatgggagattgttccgtcactgctctgggcgcatcactctgttcttcagggcaagtggcctctgtaatctgctcaggtaagagaataagggcagccagtgatgagccactcatgacggtgccttaagagtgggtgtacctaggagttcccattgtggctcagtggtaacaaactcgactggtatccatgagggtatgggtttgatccctggccttgctcaatgggttaaggatccagcattgctgtgagctgtggtataggttgcagactctgctcaggtcccatgttgctgtgattgtggtgtaggctgactgctgcagcttcaatttgacccctagcccgggaatttccataggccacacgtgcagcactaaggaaggaaaaaaagaaaaaaaaaaaaaaagagtgggtgtgcctatagtgaagaacagatgtaaaagggaagtgaaagggattcccccattctgagggattgtgagaagtgtgccagaatattaacttcatttgacttgttacagggaaagtaaacttgactttcacggacctcctagttacctggtgcttactatatgtcttctcagagtacctgattcattcccagcctggttgacccatccccctatctctatggctatgtttatccagagcacatctatctaacactccagctgatcttcctgacacagctgtggcaaccctggatcctttaaccaactgtgccaggctggagatcaaacctaagcctctgcagcaacccaagctgctgcagtcagatttttaaccccctgtgccactgtgggtatctccgatattttgtatcttctgtgactgagtggtttgctgtttgcagggaaccagagtcagacactatccccgtgcaattcatcatcctcggacccatcaagctctattatttcagaagaaaatggtgttgcctgcataggtgagaatcagtgaccaacctatgaaaatgatctcaatcctctgaaatgcattttattcatgttttatttcctctttgcagggagtggtcaacttcgcctggtcgatggaggtggtcgttgtgctgggagagtagaggtctatcatgagggctcctggggcaccatctgtgatgacagctgggacctgaatgatgcccatgtggtgtgcaaacagctgagctgtggatgggccattaatgccactggttctgctcattttggggaaggaacagggcccatttggctggatgagataaactgtaatggaaaagaatctcatatttggcaatgccactcacatggttgggggcggcacaattgcaggcataaggaggatgcaggagtcatctgctcgggtaagttctgcacatcacttcgggttacagtgatttaagaaacaactaaggtggggcaaagggtagtgaggcatatccatcagagcaaattccttgaaatacggactcagagggaaccattgtgagattgaggttcccagaggtgtggatttaatgaattagtgttacctcatgtacaaggtagtatactaccagaaagataaaaattcagaagcgagtttgcagcaaaactcatagggagaacttcttttataaataatatgaagctggatatttagtgcaccacctgatgaccactttattaataaataaagagttcctgttgtggcgcagcggaaatgaatccgacaaataatcatgagtttgcgggtttgatccctgacctcgctcagtgggttggggatctggtgttgccatgagctgtggtgtaggtcgcagatgctgcttggatcctgctttgctgtggctgtggtataggcttgtggctacagctccgatttgaccgctagcctgggaacctccatatgctgcgggggtggccctcaaaagaaaaataaataaataagtaaataaataagtagtttaaaaaggacaagaagaaatatatttggtgttatattctacagagacaaagataatcaccatgcccgattgatttttcaaggcatataaatgagacgtcatgggagcaaaaatggtcataatacaatgcccttgttttgtgtacatggtaagattttagaaagcattgtgaggtaaaaaagtgtactcagttataatatattggggaaaacagtactatgagaagtaaaaaaatctacatgccggaagttatttttttaatgtctcttttagagtcgcacatgcggcatatggaggttcccaggctaggggtcgaatcagagctatagccactggcttatggcacagccacaacaacactagatctgagccacatcagcgacctatactatagctcatggcaatgccagatccttaacctactgagccaagccatgggtcaaatccaggtcctcacggatcctaggcaaattcatttctgctgagccacgaagggaactcctcagaagtgattttgatgttactttcttttcatgacaaatctggtaaagtacatacacatagaaactgaagtgtcagaaagggaaatatttcattttaaggtaatgtatacaaaacagtggttttaccatctgagtatctcgctaaattttaactatcaaggacaattgccaaaaaaaaaaaaaaaagagagagagagagaacagaatagggttatgaagctaaaatcacagggttatgaagctaaaatcacagtaatttagggagaaaaaaatccaaagcatgtaattgataaaaggttctgagcctttgtttgagatttagaattcaacttagaaataccggtggtattttaaagcagtccataagtataaaatccaaggctaaaaaaccagaaggtatttgtagaacaaatatattttaataagctctaccaagtcatccagaagctattaaagaattactggtcactgacatagtgtacctgttttcaaggccattcttacatcagaataaagggagagcaccctctgaatcttcagaaaagatgtgaaagtgctaattctctatttcatcccagagttcatgtctctgagactgatcagtgaaaacagcagagagacctgtgcagggcgcctggaagttttttacaacggagcttggggcagcgttggcaagaatagcatgtctccagccacagtgggggtggtatgcaggcagctaggctgtgcagacagaggggacatcagccctgcatcttcagacaagacagtgtccaggcacatgtgggtggacaatgttcagtgtcctaaaggacctgacacactatggcagtgcccatcatctccatggaagaagagactggccagcccctcagaggagacatggatcacatgtgccagtgagtatccattctttagcgccactgttatcttctgatctacctaagcagaagttttataatctgtagttaatccctattctacctggatgatgggattcattctgtttaatttggtgtgcaggtattcagcatcagtgatcattttcccaaagaccatcatgctctgatggtcttctcaaaagttctaatcagttgcttcctccgtgaacagttgaggagcagagaatatgtaattcagaatttgactattgaatcatcccatttttctttcacatagtcttttgttgcactgaatataaggagagaagcagtcagaaagatcaatcctgaattatttctccattctacatctgttttaaatttcaaaaaaaaaaattgttataggtgatttacaatgtctgtcaatttctgctctacagcaaagtgacccagttatttacatatacattctgtttctcatatttttaaaccaggagatttctatctgcctggcggtttgagggaatttaacattatgcatttatgttaactttattcacctgatgttttctaagtcatactgagattcttatgcccaggatggaatacacctggtttgctggaaagacatgtgctttcataaagacgaattttggaaaaaatataaaatttaaaaggcccattaaataagcaaagttttaagagatttcaaaaaaaatttcatctctctcttttcctctttgacctcttgggcacgttcatcttctcaaatatgatcttggtgtttctgacttttcagacaaaataagacttcaagaaggaaacactaattgttctggacgtgtggagatctggtacggaggttcctggggcactgtgtgtgacgactcctgggaccttgaagatgctcaggtggtgtgccgacagctgggctgtggctcagctttggaggcaggaaaagaggccgcatttggccaggggactgggcccatatggctcaatgaagtgaagtgcaaggggaatgaaacctccttgtgggattgtcctgccagatcctggggccacagtgactgtggacacaaggaggatgctgctgtgacgtgttcaggtgagggcagagagtctggattgagcttggaagctctggcagcaaagagagggtgggcggtgacctgcattgggtaaagattggaaggtccagcctaaggatctggtggtggggggagacatgatgtttcagtctgaagaatgatgaaaacctgtgtggttacgcatgggccttcgccgaggaaagggacataactaccatgtatcctcctgcagagggaggaagaactaggggattctagttttgtgtgggaaggagcagtttacttggctcaggaggcactaaaggctcagataggaaacagagatctgttccattcttactcccagaactgattctcttctcttttctcctacagaaattgcaaagagccgagaatccctacatgccacaggtatatcaaaaagtttaagaacatgggacccattgtctgcattttgtggaatccctcttattaagacattctgggtcagaagttctgaggatttgacatttacttcagctatctgttatcttacccaagagagggatggtaactaggaacccaggtcttttagctaagacattatcacctcttgtgatgtttacttgttctcaggtcgctcatcttttgttgcacttgcaatctttggggtcattctgttggcctgtctcatcgcattcctcatttggactcagaagcgaagacagaggcagcggctctcaggtctgaacaaaattacggtctctctaatgtttctatgggagaagaagcctctctggataataaaacaaaaaaattacattcaagtatcagttggccagaaagagggaacctagaagaggtttaagcagtttctccgaaacagggaacaagaattcagagaagaaaaggcacattggctgtactgatgatacctgcactcgctatgtatgtttaatgggggacagtagagaattgatagtttagaaggagtatgcttatatggttctggatgaatcctgtatccccccaaacatttattttctcttactatatacttattactaatttaactcttctgtcaagccatgtgctaggttctgaagatggttcagacttggataaccaagtgcttttgttttcatggaatttccagtttagtggaagagataaatatgtaaacaaataaatggggggggggggggggggggggggggggggggggggggggggggggggggggggggggggggggggggggggggggggggggggggggggggggggggggggggggggggggggggggggggggggggggggggggggggggggggggggggggggggggggggggggggggggggggggggggggggggggggggggggggggggggggggggggggggggggggggggggggggggggggggggggggggggggggggggggggggggggggggggggggggggggggggggggggggggggggggggggggggggggggggggggggggggggggggggggggggggggggggggggggggggggggggggggggggggggggggggggggggggggggggggggggggggggggggggggggggggggggggggggggggggggggggggggggggggggggggggggggggggggggggggggggggggggggggggggggggggggggggggggggggggggggggggggggggggggggggggggggggggggggggggggggggggggggggggggggggggggggggggggggttggcgggcccccctcgaggtcgacggtatcgataagcttgatatcgaattcgtgagccagaggacgagactagagatggatgatgactacgttatgcttgcactgctggggaaaagcacacatagggagggaacgttttattatgacccagtccctaacctatgacctctgttatcagttttctcaggaggagagaattctgtccatcaaattcaataccgggagatgaattcttgcctgaaagcagatgaaacggatatgctaaatccctcaggtccgtgggttctttgaggggctgtagccctggggttcagatcagcagctgcagttgaggttgaggcatgctactttgcatagcagtagaaagaaatctcaactgtaataggaagcttgggatgcatatgaggaagaaaggcaagaatgaactacaaattattcttagggaagataaaaattgcagtcatggggagacctctggctgagagggccgtgattatttctgacagagggattatggagtagaatatgatggcttggaccttttttcactaaaacaagtcagtcttctcaaaggtagtttagcttttcatatatctttcacagtttcttccattcccatttcctgccattttcctttctctaacttttatttattatattttttcctaaaagtttaaattttctatatctttatcccttcagaagccatccctagtcacaggactagtctcatttcccattatgtaatgcttctttctctgtctgttgacttctatttagaaccagtgcactaaatctgcctttaggaacatacctctgctaggttgcaagaaatatcccattccccactcactctgtgaagactcaatgcttctcaatattccttacctcctgagagggacttgcctcacttctttaatccaagggactcgatttttgccaaaactaagtcaggaaaacctacataagacataggaaagacttgctgtgcttcttaaaccccactgtttgttttcctaattgtgaacagtatttttaaagttaacaagagagcttctaaggcacttgaggggagatctgatttatttcccagtaattattttcttcctttcagaaaattccactgaataagatggttttaacggatgtgggactaatttttgtgtctaaatctcttcctatttctggatgaaaaaaaggagaccactctgaagtacaatgaaaaggaaaatgggaattataacctggtgaggtgagtaggaagaatttattcatcattgctgaaaacaggtacattccttttgaaagttgagaactcctctggtattagaaaaaaaaaaagaacgtatatacacatatatttccatgtctatgtttatgtttgtaaatccatattcagaatatgcaacaactttttataactatgacttcagtccatcttttagttacatatatattctaaacaacaactattgctaagagaagctgggtaagtaaatgtgaataaatcttctaaagatattacaggaagttcctgctgcggctcagtgggttaaagacttgatgtctttgtgaagatgagggctcgagccctggcctcactcagtgagttaaggatctagcattgctgtaagctgcagcgtaggttgcagatagggctcagatccagtgttgctgtggctgtggcctcagttgcagctctgattcaacccttaggcgaggaacttccatatgcagcaaatgtggccattaaaaaaaaaaaaaacattataggagtcatttcataaaagagataagacgtttctatagttatatagtgcatactctggtaaagatagtataggatactataggaatatagaaagcttgcctatgaaaatttgggaagattgtggaaaagacatctcaaaatatggcatagaaaagaatcatatctttgaggaacagtaagtttttcattcaaaaccgtgtattgaacatacttgtggtgacaagtggtgtcctgagtactaaaaattcagtgataaaagatgctcttgacaaagacatggctgttgaatagaaggtctcactgtcaatgtgtgggaattatggacagcctatgtggacacagggaatagatgagactctaggctggaaggctgcattgagcccaataatgaatggtcctgtctgatatatttcatgctcatattttattttagggactattggggaggtggtgggttttggaagattaagctgaggcaagacacaatcagattgccttttataatttactttcaggaggaaagtctaactaaaaaaagaattcgatatcaagcttatcgataccgtcgacctcgaggaggcccgcctgcccttttggggggggggggggggggggggggggggggggggggggggggggggggggggggggggggggggggggggggggggggggggggggggggggggggggggcagcaccaattttattattggcgggaataaagagaaaaatgtaatttcaaagattgctgttggaaatgaggggtgtggtagcttttggagaaagcattctggagacttctattaattttttttttttaagtgcttcaaagatcctttgatccaacaattctactcctaaaaatttcttccatacagataaagccatttgtctgtatataacaaatagaagagaattcctttttgcagccttgttagtagtgcccccaaactggaaacaaagtgaatatcagtcagtggggtagcggctggaaaaattttagtgcacccaaccaacaaagaaaaaccatgcacaaaaattcaataaatatcatctcacttttgtgttcatgttattgaatataattaaacataatgtttacatctataaaattatcatatgtatacatgtaaagaaacattaaaacatttttaacagactgtaaacttgaggactgtgaatgacttttgattgataatctcaaacatatggatactattctgatgtaataaataatgattaaattttttccctaaagagtaatcactactgaatcgttgcctcagaatcatatggaggtgcttttaaaaaaggcatttctgcactgttgttctctggaatagaagtaattcttatgtacactgaagtttgaaaatcattgcatttaagtgttctgttcaggaaagtagtgtgctttttaatatttgtgagtgaatgagtaacacaatacattatatcacattttaatgtaattctacacatgtgcatatgaagagaaaagtaacatttttttctatttatgtctttagttcagcctttaagataccttgatgaagacctggactattgaatgagcaagaatctgcctcttacactgaagattacaatacagtcctctgtctcctggtattccaaagactgctgttgaatttctaaaaaatagattggtgaatgtgactactcaaagttgtatgtaagactttcaagggcattaaataaaaaagaatattgctgattcttgttcttgattttctgaatttctgaatctcttattgggcttctaatttaaaaaaaaatatctgggcgcccgcagatatcgaactcttgggcagtgtgaccaaacgaagacatatccaatcaagcatgcaaatggaccagcccactgtactagcacgctgtggcagccaatctgaccgagaaagcagacaaccgcagggagcaacg

SEQ ID NO: 16 - DNA, 55 bp, Sus scrofa
ggtcgccaccatggtgagcaagggcgaggagctgttcaccggggtggtgcccatc

SEQ ID NO: 17 - DNA, 54 bp, Sus scrofa
ggtcgccaccatggccatgagcaagggcgaggagctgttcaccggggtggtgcc

SEQ ID NO: 18 - DNA, 48 bp, Sus scrofa
ggtcgccaccatggtgagcaagggcgaggagctgttcaccggggtggt

SEQ ID NO: 19 - DNA, 55 bp, Sus scrofa
ggtcgccaccatggttgagcaagggcgaggagctgttcaccggggtggtgcccat

SEQ ID NO: 20 - DNA, 43 bp, Sus scrofa
tgcagggaactacagtgcggcactgtggtttccctcctggggg

SEQ ID NO: 21 - DNA, 60 bp, Sus scrofa
tgcagggaactacagtgcggcactgtaaaccactactactgtggtttccctcctgggggg

SEQ ID NO: 22 - DNA, 41 bp, Sus scrofa
tgcagggaactacagtgcggctgtggtttccctcctggggg

SEQ ID NO: 23 - DNA, 46 bp, Sus scrofa
tgcagggaactacagtgcggaactactgtggtttccctcctggggg

SEQ ID NO: 24 - DNA, 31 bp, Sus scrofa
gaaacccaggctggttggaggggacattccc

SEQ ID NO: 25 - DNA, 24 bp, Sus scrofa
gaaacccaggctggggacattccc

SEQ ID NO: 26 - DNA, 13 bp, Sus scrofa
aggggacattccc

SEQ ID NO: 27 - DNA, 13 bp, Sus scrofa
gaaacccattccc

SEQ ID NO: 28 - DNA, 31 bp, Sus scrofa
ggtcgccaccatggtgagcaagggcgaggag

SEQ ID NO: 29 - DNA, 32 bp, Sus scrofa
ggtcgccaccatggctgagcaagggcgaggag

SEQ ID NO: 30 - DNA, 29 bp, Sus scrofa
ggtcgccaccatggtgagagggcgaggag

SEQ ID NO: 31 - DNA, 32 bp, Sus scrofa
ggtcgccaccatggttgagcaagggcgaggag

SEQ ID NO: 32 - DNA, 48 bp, Sus scrofa
ggtcgccaccatggtgagcaagggcgaggagaacccaggctggttgga

SEQ ID NO: 33 - DNA, 49 bp, Sus scrofa
tgctgtgcagggaactacagtgcggcactgtggtttccctcctgggggg

SEQ ID NO: 34 - DNA, 38 bp, Sus scrofa
tgctgtgcagggaactctgtggtttccctcctgggggg

SEQ ID NO: 35 - DNA, 22 bp, Sus scrofa
ctgtggtttccctcctgggggg

SEQ ID NO: 36 - DNA, 23 bp, Sus scrofa
actgtggtttccctcctgggggg

SEQ ID NO: 37 - DNA, 50 bp, Sus scrofa
tgctgtgcagggaactacagtgcggcaactgtggtttccctcctgggggg

SEQ ID NO: 38 - DNA, 10 bp, Sus scrofa
tcctgggggg

SEQ ID NO: 39 - DNA, 8 bp, Sus scrofa
ctgggggg

SEQ ID NO: 40 - DNA, 52 bp, Sus scrofa
agagagcagagccagcgactcgcccagcgacatggggtacctgccgtttgtg

SEQ ID NO: 41 - DNA, 33 bp, Sus scrofa
agagagcagagccagcgactcgcccagcgagat

SEQ ID NO: 42 - DNA, 30 bp, Sus scrofa
agagagcagagccagcgactcgcccagcga

SEQ ID NO: 43 - DNA, 50 bp, Sus scrofa
agagccagcctcgcccagcaggggtaccatggggtacctgccgtttgtgt

SEQ ID NO: 44 - DNA, 53 bp, Sus scrofa
agagagcagagccagcgactcgcccagcgagcagtgggtacctgccgtttgtg

SEQ ID NO: 45 - DNA, 53 bp, Sus scrofa
agagagcagagccagcgactcgcccagcgatcagtgggtacctgccgtttgtg

SEQ ID NO: 46 - DNA, 53 bp, Sus scrofa
agagagcagagccagcgactcgcccagcgaacatggggtacctgccgtttgtg

SEQ ID NO: 47 - DNA, 4990 bp, Sus scrofa
tatagatgacaaggctttgtgtctgataggggccagcgaactcagtaaagagggaagatgagaaagataatggcaagaatttatccctgaagtgtagttttgacaaaccagtcacaaagaggtctaagaaattttggtcacaaagttgttttgaatcccaggcattttatttgcaatgattgcatatgttctggaaaggacatctgaacctaagaaatagttcatttgcattgtgttatattttactaaggtctgagaaataatcttgagatgagaatgaactctacttcttcagagtctggaaggaataaattatgaaaatgtattaatgcttctttaaaccatattgtatatttatctattactaaacaaaaagaagtagctctatttatttatttatttatttatttatttatgtcttttgtctctttagggccacacctgtggcatatggaggttcccaggctagaggtccaattggagatgtagcagccagcctatgccagagccaccgcaacacgggatctgagccacgtctgtgacttacaccacagctcacagcaacgcctgatcctcaacccactgagcgaggccagggatcgaacccatgtcctcatggatgctagttgggttcgttaactgctgagccatgatgggaactccaaattaattatttcttatatttgttcttcatatattcatttctatagaaagaaataaatacagattcagttaatgatggcaggtaaaagcttaacttattaatcaaaggagttaatccaggcacaaaaattcaattcatggctctctgttaaaatttaggtataggtttagcaggaagaaaaggttagtagatgcagactattacatttagaatggatggacaatgaagtcctactatacagcacagggaactatatccaatctcttgggatagaatatgatggaagacaaaatcagaacaagagagtatatatatatgtgtgtgtgtgtgtgtgtgtgtgtgtgtgtgtgtgtgtgtgtgtgactgggtcaccctgcggcacagcagaaattggcagaacattgtaaatcaactatactttaataggaaaaatacttttaagggctaaatttccaatattctaaccatgtacacagagtaaatgtcataaggatgccagtctgtgtagagattgatgtgttactagcagattcatgaaataaaggctgaggatgtagtccccaagtcacttctgagtggaagaatttctcctttgtcctggactcaaatattttaggataaaggaaaaaagaagatatttatagaagggacttgttttcaagtacttgacaaaatttcaccattaaagagaaatttgtgggagttcccatcgtggctcagtggaaacaaatccaactaggaaccatgaggttgtgggtttgatccctggcctcactcagtgggttaaggatccggtgttgccgtgagctgtggtgtaggttgcagacacggttctgatcctgcgttgctgtggctgtggctgtggtgtaggccagcagcaaacagctctgattagacccctagcctggaaacctccatatgccacaggtgcagccctaaaaagacaaaaaaagagaaaagacaaaaaaaaaaaaaaaaaaaaaaaaaaaaaaaaaaaaaaaaaaaagaacccccagaggtatttatttgtttttgccttttttcactgactgttctttgtttgtttgtttgagactgatctagaagactagagattacaagaaatatggatttggctcactctaagaaactgctttcattccaaggtttgggtctatccaaaagtggaatagaatcatatgaatactagtttatgagtatttagtgagaggaatttcaagctcaaataatgattcagcaagattaaattaaggagggaattttccttgtggctgagtgggttaaggacccaatgttgtctctgtgaggatgtaggttccatcctgggctttgctcattaggttaaggatctggcattgctgcagctcagacccagtgctgccctggttgtggcttaggccaaagctgcagctccaattcaatctctggcctgggaacctccatgtgctacaaggtgcggccttaaaaggaaaaaaaaaaaattaaatcaaggactcaagagtctttcattatttgtgttgtggaagctatatttgttttaaagtcttagttgtgtttagaaagcaagatgttcttcaactcaaatttgggagggaacttgtttcatacatttttaatggataagtggcaaaattttcatgctgaggtgatctatagtgttgtaatgcagaatatagtcagatcttgaacattttaggaagttggtgagggccaattgtgtatctgtgccatgctgataagaatgtcaagggatcacaagaattcgtgttatttgacagcagtcatctttaaaaggcatttgagaaagtccaatttcaaatgcatttcctttctttaaaagataaattgaagaaaataagtctttatttcccaagtaaattgaattgcctctcagtctgttaaaagaaactcttaccttgatgattgcgctcttaacctggcaaagattgtctttaaaatctgagctccatgtcttctgctttatttctggtgtgcctttgactccagattacagtaaatggaggactgagtatagggctaaaaagtagagagaatggatgcatattatctgtggtctccaatgtgatgaatgaagtaggcaaatactcaaaggaaagagaaagcatgctccaagaattatgggttccagaaggcaaagtcccagaattgtctccagggaaggacagggaggtctagaatcggctaagcccactgtaggcagaaaaaccaagaggcatgaatggcttccctttctcacttttcactctctggcttactcctatcatgaaggaaaatattggaatcatattctccctcaccgaaatgctatttttcagcccacaggaaacccaggctggttggaggggacattccctgctctggtcgtgttgaagtacaacatggagacacgtggggcaccgtctgtgattctgacttctctctggaggcggccagcgtgctgtgcagggaactacagtgcggcactgtggtttccctcctggggggagctcactttggagaaggaagtggacagatctgggctgaagaattccagtgtgaggggcacgagtcccacctttcactctgcccagtagcaccccgccctgacgggacatgtagccacagcagggacgtcggcgtagtctgctcaagtgagacccagggaatgtgttcactttgttcccatgccatgaagagggtagggttaggtagtcacagacatctttttaaagccctgtctccttccaggatacacacaaatccgcttggtgaatggcaagaccccatgtgaaggaagagtggagctcaacattcttgggtcctgggggtccctctgcaactctcactgggacatggaagatgcccatgttttatgccagcagcttaaatgtggagttgccctttctatcccgggaggagcaccttttgggaaaggaagtgagcaggtctggaggcacatgtttcactgcactgggactgagaagcacatgggagattgttccgtcactgctctgggcgcatcactctgttcttcagggcaagtggcctctgtaatctgctcaggtaagagaataagggcagccagtgatgagccactcatgacggtgccttaagagtgggtgtacctaggagttcccattgtggctcagtggtaacaaactcgactggtatccatgagggtatgggtttgatccctggccttgctcaatgggttaaggatccagcattgctgtgagctgtggtataggttgcagactctgctcaggtcccatgttgctgtgattgtggtgtaggctgactgctgcagcttcaatttgacccctagcccgggaatttccataggccacacgtgcagcactaaggaaggaaaaaaagaaaaaaaaaaaaaaagagtgggtgtgcctatagtgaagaacagatgtaaaagggaagtgaaagggattcccccattctgagggattgtgagaagtgtgccagaatattaacttcatttgacttgttacagggaaagtaaacttgactttcacggacctcctagttacctggtgcttactatatgtcttctcagagtacctgattcattcccagcctggttgacccatccccctatctctatggctatgtttatccagagcacatctatctaacactccagctgatcttcctgacacagctgtggcaaccctggatcctttaaccaactgtgccaggctggagatcaaacctaagcctctgcagcaacccaagctgctgcagtcagatttttaaccccctgtgccactgtgggtatctccgatattttgtatcttctgtgactgagtggtttgctgtttgcagggaaccagagtcagacactatccccgtgcaattcatcatcctcggacccatcaagctctattatttcagaagaaaatggtgttgcctgcataggtgagaatcagtgaccaacctatgaaaatgatctcaatcctctgaaatgcattttattcatgttttatttcctctttgcagggagtggtcaacttcgcctggtcgatggaggtggtcgttgtgctgggagagtagaggtctatcatgagggctcctggggcaccatctgtgatgacagctgggacctgaatgatgcccatgtggtgtgcaaacagctgagctgtggatgggccattaatgccactggttctgctcattttggggaaggaacagggcccatttggctggatgagataaactgtaatggaaaagaatctcatatttggcaatgccactcacatggttgggggcggcacaattgcaggcataaggaggatgcaggagtcatctgctcgg

SEQ ID NO: 48 - DNA, 24 bp, Artificial sequence
  Synthetic oligonucleotide
caccggaaacccaggctggttgga

SEQ ID NO: 49 - DNA, 24 bp, Artificial sequence
  Synthetic oligonucleotide
aaactccaaccagcctgggtttcc

SEQ ID NO: 50 - DNA, 24 bp, Artificial sequence
  Synthetic oligonucleotide
caccggaactacagtgcggcactg

SEQ ID NO: 51 - DNA, 24 bp, Artificial sequence
  Synthetic oligonucleotide
aaaccagtgccgcactgtagttcc

SEQ ID NO: 52 - DNA, 25 bp, Artificial sequence
  Synthetic oligonucleotide
caccgcagtagcaccccgccctgac

SEQ ID NO: 53 - DNA, 25 bp, Artificial sequence
  Synthetic oligonucleotide
aaacgtcagggcggggtgctactgc

SEQ ID NO: 54 - DNA, 25 bp, Artificial sequence
  Synthetic oligonucleotide
caccgtgtagccacagcagggacgt

SEQ ID NO: 55 - DNA, 25 bp, Artificial sequence
  Synthetic oligonucleotide
aaacacgtccctgctgtggctacac

SEQ ID NO: 56 - DNA, 25 bp, Artificial sequence
  Synthetic oligonucleotide
caccgccagcctcgcccagcgacat

SEQ ID NO: 57 - DNA, 25 bp, Artificial sequence
  Synthetic oligonucleotide
aaacatgtcgctgggcgaggctggc

SEQ ID NO: 58 - DNA, 25 bp, Artificial sequence
  Synthetic oligonucleotide
caccgcagctgcagcatatatttaa

SEQ ID NO: 59 - DNA, 25 bp, Artificial sequence
  Synthetic oligonucleotide
aaacttaaatatatgctgcagctgc

SEQ ID NO: 60 - DNA, 25 bp, Artificial sequence
  Synthetic oligonucleotide
caccgctttcatttatctgaactca

SEQ ID NO: 61 - DNA, 25 bp, Artificial sequence
  Synthetic oligonucleotide
aaactgagttcagataaatgaaagc

SEQ ID NO: 62 - DNA, 25 bp, Artificial sequence
  Synthetic oligonucleotide
caccgttatctgaactcagggtccc

SEQ ID NO: 63 - DNA, 25 bp, Artificial sequence
  Synthetic oligonucleotide
aaacgggaccctgagttcagataac

SEQ ID NO: 64 - DNA, 25 bp, Artificial sequence
  Synthetic oligonucleotide
caccgctcctcgcccttgctcacca

SEQ ID NO: 65 - DNA, 25 bp, Artificial sequence
  Synthetic oligonucleotide
aaactggtgagcaagggcgaggagc

SEQ ID NO: 66 - DNA, 25 bp, Artificial sequence
  Synthetic oligonucleotide
caccggaccaggatgggcaccaccc

SEQ ID NO: 67 - DNA, 25 bp, Artificial sequence
  Synthetic oligonucleotide
aaacgggtggtgcccatcctggtcc

SEQ ID NO: 68 - DNA, 24 bp, Artificial sequence
  Synthetic oligonucleotide
ttgttggaaggctcactgtccttg

SEQ ID NO: 69 - DNA, 20 bp, Artificial sequence
  Synthetic oligonucleotide
acaactaaggtggggcaaag

SEQ ID NO: 70 - DNA, 24 bp, Artificial sequence
  Synthetic oligonucleotide
ttgttggaaggctcactgtccttg

SEQ ID NO: 71 - DNA, 23 bp, Artificial sequence
  Synthetic oligonucleotide
ggagctcaacattcttgggtcct

SEQ ID NO: 72 - DNA, 23 bp, Artificial sequence
  Synthetic oligonucleotide
ggcaaaattttcatgctgaggtg

SEQ ID NO: 73 - DNA, 23 bp, Artificial sequence
  Synthetic oligonucleotide
gcacatcacttcgggttacagtg

SEQ ID NO: 74 - DNA, 23 bp, Artificial sequence
  Synthetic oligonucleotide
cccaagtatcttcagttctgcag

SEQ ID NO: 75 - DNA, 23 bp, Artificial sequence
  Synthetic oligonucleotide
tacaggtaggagagcctgttttg

SEQ ID NO: 76 - DNA, 23 bp, Artificial sequence
  Synthetic oligonucleotide
cccaagtatcttcagttctgcag

SEQ ID NO: 77 - DNA, 23 bp, Artificial sequence
  Synthetic oligonucleotide
ctcaaaaggatgtaaaccctgga

SEQ ID NO: 78 - DNA, 22 bp, Artificial sequence
  Synthetic oligonucleotide
tgttgatgtggtttgtttgccc

SEQ ID NO: 79 - DNA, 23 bp, Artificial sequence
  Synthetic oligonucleotide
tacaggtaggagagcctgttttg

SEQ ID NO: 80 - DNA, 23 bp, Artificial sequence
  Synthetic oligonucleotide
ggaggtctagaatcggctaagcc

SEQ ID NO: 81 - DNA, 20 bp, Artificial sequence
  Synthetic oligonucleotide
ggctacatgtcccgtcaggg

SEQ ID NO: 82 - DNA, 21 bp, Artificial sequence
  Synthetic oligonucleotide
gcaggccactaggcagatgaa

SEQ ID NO: 83 - DNA, 23 bp, Artificial sequence
  Synthetic oligonucleotide
gagctgacacccaagaagttcct

SEQ ID NO: 84 - DNA, 22 bp, Artificial sequence
  Synthetic oligonucleotide
ggctctagagcctctgctaacc

SEQ ID NO: 85 - DNA, 22 bp, Artificial sequence
  Synthetic oligonucleotide
ggacttgaagaagtcgtgctgc

SEQ ID NO: 86 - DNA, 44 bp, Artificial sequence
  Synthetic oligonucleotide
taatacgactcactatagggagaatggactataaggaccacgac

SEQ ID NO: 87 - DNA, 21 bp, Artificial sequence
  Synthetic oligonucleotide
gcgagctctaggaattcttac

SEQ ID NO: 88 - DNA, 40 bp, Artificial sequence
  Synthetic oligonucleotide
ttaatacgactcactataggctcctcgcccttgctcacca

SEQ ID NO: 89 - DNA, 20 bp, Artificial sequence
  Synthetic oligonucleotide
aaaagcaccgactcggtgcc

SEQ ID NO: 90 - DNA, 38 bp, Artificial sequence
  Synthetic oligonucleotide
ttaatacgactcactataggaaacccaggctggttgga

SEQ ID NO: 91 - DNA, 20 bp, Artificial sequence
  Synthetic oligonucleotide
aaaagcaccgactcggtgcc

SEQ ID NO: 92 - DNA, 38 bp, Artificial sequence
  Synthetic oligonucleotide
ttaatacgactcactataggaactacagtgcggcactg

SEQ ID NO: 93 - DNA, 20 bp, Artificial sequence
  Synthetic oligonucleotide
aaaagcaccgactcggtgcc

SEQ ID NO: 94 - DNA, 40 bp, Artificial sequence
  Synthetic oligonucleotide
ttaatacgactcactataggccagcctcgcccagcgacat

SEQ ID NO: 95 - DNA, 20 bp, Artificial sequence
  Synthetic oligonucleotide
aaaagcaccgactcggtgcc

SEQ ID NO: 96 - DNA, 40 bp, Artificial sequence
  Synthetic oligonucleotide
ttaatacgactcactataggcagctgcagcatatatttaa

SEQ ID NO: 97 - DNA, 20 bp, Artificial sequence
  Synthetic oligonucleotide
aaaagcaccgactcggtgcc

SEQ ID NO: 98 - DNA, 3484 bp, Sus scrofa
tatagatgacaaggctttgtgtctgataggggccagcgaactcagtaaagagggaagatgagaaagataatggcaagaatttatccctgaagtgtagttttgacaaaccagtcacaaagaggtctaagaaattttggtcacaaagttgttttgaatcccaggcattttatttgcaatgattgcatatgttctggaaaggacatctgaacctaagaaatagttcatttgcattgtgttatattttactaaggtctgagaaataatcttgagatgagaatgaactctacttcttcagagtctggaaggaataaattatgaaaatgtattaatgcttctttaaaccatattgtatatttatctattactaaacaaaaagaagtagctctatttatttatttatttatttatttatttatgtcttttgtctctttagggccacacctgtggcatatggaggttcccaggctagaggtccaattggagatgtagcagccagcctatgccagagccaccgcaacacgggatctgagccacgtctgtgacttacaccacagctcacagcaacgcctgatcctcaacccactgagcgaggccagggatcgaacccatgtcctcatggatgctagttgggttcgttaactgctgagccatgatgggaactccaaattaattatttcttatatttgttcttcatatattcatttctatagaaagaaataaatacagattcagttaatgatggcaggtaaaagcttaacttattaatcaaaggagttaatccaggcacaaaaattcaattcatggctctctgttaaaatttaggtataggtttagcaggaagaaaaggttagtagatgcagactattacatttagaatggatggacaatgaagtcctactatacagcacagggaactatatccaatctcttgggatagaatatgatggaagacaaaatcagaacaagagagtatatatatatgtgtgtgtgtgtgtgtgtgtgtgtgtgtgtgtgtgtgtgtgtgtgactgggtcaccctgcggcacagcagaaattggcagaacattgtaaatcaactatactttaataggaaaaatacttttaagggctaaatttccaatattctaaccatgtacacagagtaaatgtcataaggatgccagtctgtgtagagattgatgtgttactagcagattcatgaaataaaggctgaggatgtagtccccaagtcacttctgagtggaagaatttctcctttgtcctggactcaaatattttaggataaaggaaaaaagaagatatttatagaagggacttgttttcaagtacttgacaaaatttcaccattaaagagaaatttgtgggagttcccatcgtggctcagtggaaacaaatccaactaggaaccatgaggttgtgggtttgatccctggcctcactcagtgggttaaggatccggtgttgccgtgagctgtggtgtaggttgcagacacggttctgatcctgcgttgctgtggctgtggcacattccctgctctggtcgtgttgaagtacaacatggagacacgtggggcaccgtctgtgattctgacttctctctggaggcggccagcgtgctgtgcagggaactacagtgcggcactgtggtttccctcctggggggagctcactttggagaaggaagtggacagatctgggctgaagaattccagtgtgaggggcacgagtcccacctttcactctgcccagtagcaccccgccctgacgggacatgtagccacagcagggacgtcggcgtagtctgctcaagtgagacccagggaatgtgttcactttgttcccatgccatgaagagggtagggttaggtagtcacagacatctttttaaagccctgtctccttccaggatacacacaaatccgcttggtgaatggcaagaccccatgtgaaggaagagtggagctcaacattcttgggtcctgggggtccctctgcaactctcactgggacatggaagatgcccatgttttatgccagcagcttaaatgtggagttgccctttctatcccgggaggagcaccttttgggaaaggaagtgagcaggtctggaggcacatgtttcactgcactgggactgagaagcacatgggagattgttccgtcactgctctgggcgcatcactctgttcttcagggcaagtggcctctgtaatctgctcaggtaagagaataagggcagccagtgatgagccactcatgacggtgccttaagagtgggtgtacctaggagttcccattgtggctcagtggtaacaaactcgactggtatccatgagggtatgggtttgatccctggccttgctcaatgggttaaggatccagcattgctgtgagctgtggtataggttgcagactctgctcaggtcccatgttgctgtgattgtggtgtaggctgactgctgcagcttcaatttgacccctagcccgggaatttccataggccacacgtgcagcactaaggaaggaaaaaaagaaaaaaaaaaaaaaagagtgggtgtgcctatagtgaagaacagatgtaaaagggaagtgaaagggattcccccattctgagggattgtgagaagtgtgccagaatattaacttcatttgacttgttacagggaaagtaaacttgactttcacggacctcctagttacctggtgcttactatatgtcttctcagagtacctgattcattcccagcctggttgacccatccccctatctctatggctatgtttatccagagcacatctatctaacactccagctgatcttcctgacacagctgtggcaaccctggatcctttaaccaactgtgccaggctggagatcaaacctaagcctctgcagcaacccaagctgctgcagtcagatttttaaccccctgtgccactgtgggtatctccgatattttgtatcttctgtgactgagtggtttgctgtttgcagggaaccagagtcagacactatccccgtgcaattcatcatcctcggacccatcaagctctattatttcagaagaaaatggtgttgcctgcataggtgagaatcagtgaccaacctatgaaaatgatctcaatcctctgaaatgcattttattcatgttttatttcctctttgcagggagtggtcaacttcgcctggtcgatggaggtggtcgttgtgctgggagagtagaggtctatcatgagggctcctggggcaccatctgtgatgacagctgggacctgaatgatgcccatgtggtgtgcaaacagctgagctgtggatgggccattaatgccactggttctgctcattttggggaaggaacagggcccatttggctggatgagataaactgtaatggaaaagaatctcatatttggcaatgccactcacatggttgggggcggcacaattgcaggcataaggaggatgcaggagtcatctgctcgg

SEQ ID NO: 99 - DNA, 4997 bp, Sus scrofa
tatagatgacaaggctttgtgtctgataggggccagcgaactcagtaaagagggaagatgagaaagataatggcaagaatttatccctgaagtgtagttttgacaaaccagtcacaaagaggtctaagaaattttggtcacaaagttgttttgaatcccaggcattttatttgcaatgattgcatatgttctggaaaggacatctgaacctaagaaatagttcatttgcattgtgttatattttactaaggtctgagaaataatcttgagatgagaatgaactctacttcttcagagtctggaaggaataaattatgaaaatgtattaatgcttctttaaaccatattgtatatttatctattactaaacaaaaagaagtagctctatttatttatttatttatttatttatttatgtcttttgtctctttagggccacacctgtggcatatggaggttcccaggctagaggtccaattggagatgtagcagccagcctatgccagagccaccgcaacacgggatctgagccacgtctgtgacttacaccacagctcacagcaacgcctgatcctcaacccactgagcgaggccagggatcgaacccatgtcctcatggatgctagttgggttcgttaactgctgagccatgatgggaactccaaattaattatttcttatatttgttcttcatatattcatttctatagaaagaaataaatacagattcagttaatgatggcaggtaaaagcttaacttattaatcaaaggagttaatccaggcacaaaaattcaattcatggctctctgttaaaatttaggtataggtttagcaggaagaaaaggttagtagatgcagactattacatttagaatggatggacaatgaagtcctactatacagcacagggaactatatccaatctcttgggatagaatatgatggaagacaaaatcagaacaagagagtatatatatatgtgtgtgtgtgtgtgtgtgtgtgtgtgtgtgtgtgtgtgtgtgtgactgggtcaccctgcggcacagcagaaattggcagaacattgtaaatcaactatactttaataggaaaaatacttttaagggctaaatttccaatattctaaccatgtacacagagtaaatgtcataaggatgccagtctgtgtagagattgatgtgttactagcagattcatgaaataaaggctgaggatgtagtccccaagtcacttctgagtggaagaatttctcctttgtcctggactcaaatattttaggataaaggaaaaaagaagatatttatagaagggacttgttttcaagtacttgacaaaatttcaccattaaagagaaatttgtgggagttcccatcgtggctcagtggaaacaaatccaactaggaaccatgaggttgtgggtttgatccctggcctcactcagtgggttaaggatccggtgttgccgtgagctgtggtgtaggttgcagacacggttctgatcctgcgttgctgtggctgtggctgtggtgtaggccagcagcaaacagctctgattagacccctagcctggaaacctccatatgccacaggtgcagccctaaaaagacaaaaaaagagaaaagacaaaaaaaaaaaaaaaaaaaaaaaaaaaaaaaaaaaaaaaaaaaagaacccccagaggtatttatttgtttttgccttttttcactgactgttctttgtttgtttgtttgagactgatctagaagactagagattacaagaaatatggatttggctcactctaagaaactgctttcattccaaggtttgggtctatccaaaagtggaatagaatcatatgaatactagtttatgagtatttagtgagaggaatttcaagctcaaataatgattcagcaagattaaattaaggagggaattttccttgtggctgagtgggttaaggacccaatgttgtctctgtgaggatgtaggttccatcctgggctttgctcattaggttaaggatctggcattgctgcagctcagacccagtgctgccctggttgtggcttaggccaaagctgcagctccaattcaatctctggcctgggaacctccatgtgctacaaggtgcggccttaaaaggaaaaaaaaaaaattaaatcaaggactcaagagtctttcattatttgtgttgtggaagctatatttgttttaaagtcttagttgtgtttagaaagcaagatgttcttcaactcaaatttgggagggaacttgtttcatacatttttaatggataagtggcaaaattttcatgctgaggtgatctatagtgttgtaatgcagaatatagtcagatcttgaacattttaggaagttggtgagggccaattgtgtatctgtgccatgctgataagaatgtcaagggatcacaagaattcgtgttatttgacagcagtcatctttaaaaggcatttgagaaagtccaatttcaaatgcatttcctttctttaaaagataaattgaagaaaataagtctttatttcccaagtaaattgaattgcctctcagtctgttaaaagaaactcttaccttgatgattgcgctcttaacctggcaaagattgtctttaaaatctgagctccatgtcttctgctttatttctggtgtgcctttgactccagattacagtaaatggaggactgagtatagggctaaaaagtagagagaatggatgcatattatctgtggtctccaatgtgatgaatgaagtaggcaaatactcaaaggaaagagaaagcatgctccaagaattatgggttccagaaggcaaagtcccagaattgtctccagggaaggacagggaggtctagaatcggctaagcccactgtaggcagaaaaaccaagaggcatgaatggcttccctttctcacttttcactctctggcttactcctatcatgaaggaaaatattggaatcatattctccctcaccgaaatgctatttttcagcccacaggaaacccaggctggttggaggggacattccctgctctggtcgtgttgaagtacaacatggagacacgtggggcaccgtctgtgattctgacttctctctggaggcggccagcgtgctgtgcagggaactacagtgcggctactactactgtggtttccctcctggggggagctcactttggagaaggaagtggacagatctgggctgaagaattccagtgtgaggggcacgagtcccacctttcactctgcccagtagcaccccgccctgacgggacatgtagccacagcagggacgtcggcgtagtctgctcaagtgagacccagggaatgtgttcactttgttcccatgccatgaagagggtagggttaggtagtcacagacatctttttaaagccctgtctccttccaggatacacacaaatccgcttggtgaatggcaagaccccatgtgaaggaagagtggagctcaacattcttgggtcctgggggtccctctgcaactctcactgggacatggaagatgcccatgttttatgccagcagcttaaatgtggagttgccctttctatcccgggaggagcaccttttgggaaaggaagtgagcaggtctggaggcacatgtttcactgcactgggactgagaagcacatgggagattgttccgtcactgctctgggcgcatcactctgttcttcagggcaagtggcctctgtaatctgctcaggtaagagaataagggcagccagtgatgagccactcatgacggtgccttaagagtgggtgtacctaggagttcccattgtggctcagtggtaacaaactcgactggtatccatgagggtatgggtttgatccctggccttgctcaatgggttaaggatccagcattgctgtgagctgtggtataggttgcagactctgctcaggtcccatgttgctgtgattgtggtgtaggctgactgctgcagcttcaatttgacccctagcccgggaatttccataggccacacgtgcagcactaaggaaggaaaaaaagaaaaaaaaaaaaaaagagtgggtgtgcctatagtgaagaacagatgtaaaagggaagtgaaagggattcccccattctgagggattgtgagaagtgtgccagaatattaacttcatttgacttgttacagggaaagtaaacttgactttcacggacctcctagttacctggtgcttactatatgtcttctcagagtacctgattcattcccagcctggttgacccatccccctatctctatggctatgtttatccagagcacatctatctaacactccagctgatcttcctgacacagctgtggcaaccctggatcctttaaccaactgtgccaggctggagatcaaacctaagcctctgcagcaacccaagctgctgcagtcagatttttaaccccctgtgccactgtgggtatctccgatattttgtatcttctgtgactgagtggtttgctgtttgcagggaaccagagtcagacactatccccgtgcaattcatcatcctcggacccatcaagctctattatttcagaagaaaatggtgttgcctgcataggtgagaatcagtgaccaacctatgaaaatgatctcaatcctctgaaatgcattttattcatgttttatttcctctttgcagggagtggtcaacttcgcctggtcgatggaggtggtcgttgtgctgggagagtagaggtctatcatgagggctcctggggcaccatctgtgatgacagctgggacctgaatgatgcccatgtggtgtgcaaacagctgagctgtggatgggccattaatgccactggttctgctcattttggggaaggaacagggcccatttggctggatgagataaactgtaatggaaaagaatctcatatttggcaatgccactcacatggttgggggcggcacaattgcaggcataaggaggatgcaggagtcatctgctcgg

SEQ ID NO: 100 - DNA, 3710 bp, Sus scrofa
tatagatgacaaggctttgtgtctgataggggccagcgaactcagtaaagagggaagatgagaaagataatggcaagaatttatccctgaagtgtagttttgacaaaccagtcacaaagaggtctaagaaattttggtcacaaagttgttttgaatcccaggcattttatttgcaatgattgcatatgttctggaaaggacatctgaacctaagaaatagttcatttgcattgtgttatattttactaaggtctgagaaataatcttgagatgagaatgaactctacttcttcagagtctggaaggaataaattatgaaaatgtattaatgcttctttaaaccatattgtatatttatctattactaaacaaaaagaagtagctctatttatttatttatttatttatttatttatgtcttttgtctctttagggccacacctgtggcatatggaggttcccaggctagaggtccaattggagatgtagcagccagcctatgccagagccaccgcaacacgggatctgagccacgtctgtgacttacaccacagctcacagcaacgcctgatcctcaacccactgagcgaggccagggatcgaacccatgtcctcatggatgctagttgggttcgttaactgctgagccatgatgggaactccaaattaattatttcttatatttgttcttcatatattcatttctatagaaagaaataaatacagattcagttaatgatggcaggtaaaagcttaacttattaatcaaaggagttaatccaggcacaaaaattcaattcatggctctctgttaaaatttaggtataggtttagcaggaagaaaaggttagtagatgcagactattacatttagaatggatggacaatgaagtcctactatacagcacagggaactatatccaatctcttgggatagaatatgatggaagacaaaatcagaacaagagagtatatatatatgtgtgtgtgtgtgtgtgtgtgtgtgtgtgtgtgtgtgtgtgtgtgactgggtcaccctgcggcacagcagaaattggcagaacattgtaaatcaactatactttaataggaaaaatacttttaagggctaaatttccaatattctaaccatgtacacagagtaaatgtcataaggatgccagtctgtgtagagattgatgtgttactagcagattcatgaaataaaggctgaggatgtagtccccaagtcacttctgagtggaagaatttctcctttgtcctggactcaaatattttaggataaaggaaaaaagaagatatttatagaagggacttgttttcaagtacttgacaaaatttcaccattaaagagaaatttgtgggagttcccatcgtggctcagtggaaacaaatccaactaggaaccatgaggttgtgggtttgatccctggcctcactcagtgggttaaggatccggtgttgccgtgagctgtggtgtaggttgcagacacggttctgatcctgcgttgctgtggctgtggctgtggtgtaggccagcagcaaacagctctgattagacccctagcctggaaacctccatatgccacaggtgcagccctaaaaagacaaaaaaagagaaaagacaaaaaaaaaaaaaaaaaaaaaaaaaaaaaaaaaaaaaaaaaaaagaacccccagaggtatttatttgtttttgccttttttcactgactgttctttgtttgtttgtttgagactgatctagaagactagagattacaagaaatatggatttggctcactctaagaaactgctttcattccaaggtttgggtctatccaaaagtggaatagaatcatatgaatactagtttatgagtatttagtgagaggaatttcaagctcaaataatgattcagcaagattaaattaaggagggaattttccttgtggctgagtgggttaaggacccaatgttgtctctgtgaggatgtaggttccatcctgggctttgctcattaggttaaggatctggcattgctgcagctcagacccagtgctgccctggttgtggcttaggccaaagctgcagctccaattcaatctctggcctgggaacctccatgtgctacaaggtgcggccttaaaaggaaaaaaaaaaaattaaatcaaggactcaagagtctttcattatttgtgttgtggaagctatatttgttttaaagtcttagttgtgtttagaaagcaagatgttcttcaactcaaatttgggagggaacttgtttcatacatttttaatggataagtggcaaaattttcatgctgaggtgatctatagtgttgtaatgcagaatatagtcagatcttgaacattttaggaagttggtgagggccaattgtgtatctgtgccatgctgataagaatgtcaagggatcacaagaattcgtgttatttgacagcagtcatctttaaaaggcatttgagaaagtccaatttcaaatgcatttcctttctttaaaagataaattgaagaaaataagtctttatttcccaagtaaattgaattgcctctcagtctgttaaaagaaactcttaccttgatgattgcgctcttaacctggcaaagattgtctttaaaatctgagctccatgtcttctgctttatttctggtgtgcctttgactccagattacagtaaatggaggactgagtatagggctaaaaagtagagagaatggatgcatattatctgtggtctccaatgtgatgaatgaagtaggcaaatactcaaaggaaagagaaagcatgctccaagaattatgggttccagaagggaaagggattcccccattctgagggattgtgagaagtgtgccagaatattaacttcatttgacttgttacagggaaagtaaacttgactttcacggacctcctagttacctggtgcttactatatgtcttctcagagtacctgattcattcccagcctggttgacccatccccctatctctatggctatgtttatccagagcacatctatctaacactccagctgatcttcctgacacagctgtggcaaccctggatcctttaaccaactgtgccaggctggagatcaaacctaagcctctgcagcaacccaagctgctgcagtcagatttttaaccccctgtgccactgtgggtatctccgatattttgtatcttctgtgactgagtggtttgctgtttgcagggaaccagagtcagacactatccccgtgcaattcatcatcctcggacccatcaagctctattatttcagaagaaaatggtgttgcctgcataggtgagaatcagtgaccaacctatgaaaatgatctcaatcctctgaaatgcattttattcatgttttatttcctctttgcagggagtggtcaacttcgcctggtcgatggaggtggtcgttgtgctgggagagtagaggtctatcatgagggctcctggggcaccatctgtgatgacagctgggacctgaatgatgcccatgtggtgtgcaaacagctgagctgtggatgggccattaatgccactggttctgctcattttggggaaggaacagggcccatttggctggatgagataaactgtaatggaaaagaatctcatatttggcaatgccactcacatggttgggggcggcacaattgcaggcataaggaggatgcaggagtcatctgctcgg

SEQ ID NO: 101 - DNA, 3617 bp, Sus scrofa
tatagatgacaaggctttgtgtctgataggggccagcgaactcagtaaagagggaagatgagaaagataatggcaagaatttatccctgaagtgtagttttgacaaaccagtcacaaagaggtctaagaaattttggtcacaaagttgttttgaatcccaggcattttatttgcaatgattgcatatgttctggaaaggacatctgaacctaagaaatagttcatttgcattgtgttatattttactaaggtctgagaaataatcttgagatgagaatgaactctacttcttcagagtctggaaggaataaattatgaaaatgtattaatgcttctttaaaccatattgtatatttatctattactaaacaaaaagaagtagctctatttatttatttatttatttatttatttatgtcttttgtctctttagggccacacctgtggcatatggaggttcccaggctagaggtccaattggagatgtagcagccagcctatgccagagccaccgcaacacgggatctgagccacgtctgtgacttacaccacagctcacagcaacgcctgatcctcaacccactgagcgaggccagggatcgaacccatgtcctcatggatgctagttgggttcgttaactgctgagccatgatgggaactccaaattaattatttcttatatttgttcttcatatattcatttctatagaaagaaataaatacagattcagttaatgatggcaggtaaaagcttaacttattaatcaaaggagttaatccaggcacaaaaattcaattcatggctctctgttaaaatttaggtataggtttagcaggaagaaaaggttagtagatgcagactattacatttagaatggatggacaatgaagtcctactatacagcacagggaactatatccaatctcttgggatagaatatgatggaagacaaaatcagaacaagagagtatatatatatgtgtgtgtgtgtgtgtgtgtgtgtgtgtgtgtgtgtgtgtgtgtgactgggtcaccctgcggcacagcagaaattggcagaacattgtaaatcaactatactttaataggaaaaatacttttaagggctaaatttccaatattctaaccatgtacacagagtaaatgtcataaggatgccagtctgtgtagagattgatgtgttactagcagattcatgaaataaaggctgaggatgtagtccccaagtcacttctgagtggaagaatttctcctttgtcctggactcaaatattttaggataaaggaaaaaagaagatatttatagaagggacttgttttcaagtacttgacaaaatttcaccattaaagagaaatttgtgggagttcccatcgtggctcagtggaaacaaatccaactaggaaccatgaggttgtgggtttgatccctggcctcactcagtgggttaaggatccggtgttgccgtgagctgtggtgtaggttgcagacacggttctgatcctgcgttgctgtggctgtggctgtggtgtaggccagcagcaaacagctctgattagacccctagcctggaaacctccatatgccacaggtgcagccctaaaaagacaaaaaaagagaaaagacaaaaaaaaaaaaaaaaaaaaaaaaaaaaaaaaaaaaaaaaaaaagaacccccagaggtatttatttgtttttgccttttttcactgactgttctttgtttgtttgtttgagactgatctagaagactagagattacaagaaatatggatttggctcactctaagaaactgctttcattccaaggtttgggtctatccaaaagtggaatagaatcatatgaatactagtttatgagtatttagtgagaggaatttcaagctcaaataatgattcagcaagattaaattaaggagggaattttccttgtggctgagtgggttaaggacccaatgttgtctctgtgaggatgtaggttccatcctgggctttgctcattaggttaaggatctggcattgctgcagctcagacccagtgctgccctggttgtggcttaggccaaagctgcagctccaattcaatctctggcctgggaacctccatgtgctacaaggtgcggccttaaaaggaaaaaaaaaaaattaaatcaaggactcaagagtctttcattatttgtgttgtggaagctatatttgttttaaagtcttagttgtgtttagaaagcaagatgttcttcaactcaaatttgggagggaacttgtttcatacatttttaatggataagtggcaaaattttcatgctgaggtgatctatagtgttgtaatgcagaatatagtcagatcttgaacattttaggaagttggtgagggccaattgtgtatctgtgccatgctgataagaatgtcaagggatcacaagaattcgtgttatttgacagcagtcatctttaaaaggcatttgagaaagtccaatttcaaatgcatttcctttctttaaaagataaattgaagaaaataagtctttatttcccaagtaaattgaattgcctctcagtctgttaaaagaaactcttaccttgatgattgcgctcttaacctggcaaagattgtctttaaaatctgagctccatgtcttctgctttatttctggtgtgcctttgactccagattacagtaaatggaggactgagtatagggctaaaaagtagagagaatggattgaaagggattcccccattctgagggattgtgagaagtgtgccagaatattaacttcatttgacttgttacagggaaagtaaacttgactttcacggacctcctagttacctggtgcttactatatgtcttctcagagtacctgattcattcccagcctggttgacccatccccctatctctatggctatgtttatccagagcacatctatctaacactccagctgatcttcctgacacagctgtggcaaccctggatcctttaaccaactgtgccaggctggagatcaaacctaagcctctgcagcaacccaagctgctgcagtcagatttttaaccccctgtgccactgtgggtatctccgatattttgtatcttctgtgactgagtggtttgctgtttgcagggaaccagagtcagacactatccccgtgcaattcatcatcctcggacccatcaagctctattatttcagaagaaaatggtgttgcctgcataggtgagaatcagtgaccaacctatgaaaatgatctcaatcctctgaaatgcattttattcatgttttatttcctctttgcagggagtggtcaacttcgcctggtcgatggaggtggtcgttgtgctgggagagtagaggtctatcatgagggctcctggggcaccatctgtgatgacagctgggacctgaatgatgcccatgtggtgtgcaaacagctgagctgtggatgggccattaatgccactggttctgctcattttggggaaggaacagggcccatttggctggatgagataaactgtaatggaaaagaatctcatatttggcaatgccactcacatggttgggggcggcacaattgcaggcataaggaggatgcaggagtcatctgctcgg

SEQ ID NO: 102 - DNA, 4979 bp, Sus scrofa
tatagatgacaaggctttgtgtctgataggggccagcgaactcagtaaagagggaagatgagaaagataatggcaagaatttatccctgaagtgtagttttgacaaaccagtcacaaagaggtctaagaaattttggtcacaaagttgttttgaatcccaggcattttatttgcaatgattgcatatgttctggaaaggacatctgaacctaagaaatagttcatttgcattgtgttatattttactaaggtctgagaaataatcttgagatgagaatgaactctacttcttcagagtctggaaggaataaattatgaaaatgtattaatgcttctttaaaccatattgtatatttatctattactaaacaaaaagaagtagctctatttatttatttatttatttatttatttatgtcttttgtctctttagggccacacctgtggcatatggaggttcccaggctagaggtccaattggagatgtagcagccagcctatgccagagccaccgcaacacgggatctgagccacgtctgtgacttacaccacagctcacagcaacgcctgatcctcaacccactgagcgaggccagggatcgaacccatgtcctcatggatgctagttgggttcgttaactgctgagccatgatgggaactccaaattaattatttcttatatttgttcttcatatattcatttctatagaaagaaataaatacagattcagttaatgatggcaggtaaaagcttaacttattaatcaaaggagttaatccaggcacaaaaattcaattcatggctctctgttaaaatttaggtataggtttagcaggaagaaaaggttagtagatgcagactattacatttagaatggatggacaatgaagtcctactatacagcacagggaactatatccaatctcttgggatagaatatgatggaagacaaaatcagaacaagagagtatatatatatgtgtgtgtgtgtgtgtgtgtgtgtgtgtgtgtgtgtgtgtgtgtgactgggtcaccctgcggcacagcagaaattggcagaacattgtaaatcaactatactttaataggaaaaatacttttaagggctaaatttccaatattctaaccatgtacacagagtaaatgtcataaggatgccagtctgtgtagagattgatgtgttactagcagattcatgaaataaaggctgaggatgtagtccccaagtcacttctgagtggaagaatttctcctttgtcctggactcaaatattttaggataaaggaaaaaagaagatatttatagaagggacttgttttcaagtacttgacaaaatttcaccattaaagagaaatttgtgggagttcccatcgtggctcagtggaaacaaatccaactaggaaccatgaggttgtgggtttgatccctggcctcactcagtgggttaaggatccggtgttgccgtgagctgtggtgtaggttgcagacacggttctgatcctgcgttgctgtggctgtggctgtggtgtaggccagcagcaaacagctctgattagacccctagcctggaaacctccatatgccacaggtgcagccctaaaaagacaaaaaaagagaaaagacaaaaaaaaaaaaaaaaaaaaaaaaaaaaaaaaaaaaaaaaaaaagaacccccagaggtatttatttgtttttgccttttttcactgactgttctttgtttgtttgtttgagactgatctagaagactagagattacaagaaatatggatttggctcactctaagaaactgctttcattccaaggtttgggtctatccaaaagtggaatagaatcatatgaatactagtttatgagtatttagtgagaggaatttcaagctcaaataatgattcagcaagattaaattaaggagggaattttccttgtggctgagtgggttaaggacccaatgttgtctctgtgaggatgtaggttccatcctgggctttgctcattaggttaaggatctggcattgctgcagctcagacccagtgctgccctggttgtggcttaggccaaagctgcagctccaattcaatctctggcctgggaacctccatgtgctacaaggtgcggccttaaaaggaaaaaaaaaaaattaaatcaaggactcaagagtctttcattatttgtgttgtggaagctatatttgttttaaagtcttagttgtgtttagaaagcaagatgttcttcaactcaaatttgggagggaacttgtttcatacatttttaatggataagtggcaaaattttcatgctgaggtgatctatagtgttgtaatgcagaatatagtcagatcttgaacattttaggaagttggtgagggccaattgtgtatctgtgccatgctgataagaatgtcaagggatcacaagaattcgtgttatttgacagcagtcatctttaaaaggcatttgagaaagtccaatttcaaatgcatttcctttctttaaaagataaattgaagaaaataagtctttatttcccaagtaaattgaattgcctctcagtctgttaaaagaaactcttaccttgatgattgcgctcttaacctggcaaagattgtctttaaaatctgagctccatgtcttctgctttatttctggtgtgcctttgactccagattacagtaaatggaggactgagtatagggctaaaaagtagagagaatggatgcatattatctgtggtctccaatgtgatgaatgaagtaggcaaatactcaaaggaaagagaaagcatgctccaagaattatgggttccagaaggcaaagtcccagaattgtctccagggaaggacagggaggtctagaatcggctaagcccactgtaggcagaaaaaccaagaggcatgaatggcttccctttctcacttttcactctctggcttactcctatcatgaaggaaaatattggaatcatattctccctcaccgaaatgctatttttcagcccacaggaaacccaggctggttggaggggacattccctgctctggtcgtgttgaagtacaacatggagacacgtggggcaccgtctgtgattctgacttctctctggaggcggccagcgtgctgtgcagggaactctgtggtttccctcctggggggagctcactttggagaaggaagtggacagatctgggctgaagaattccagtgtgaggggcacgagtcccacctttcactctgcccagtagcaccccgccctgacgggacatgtagccacagcagggacgtcggcgtagtctgctcaagtgagacccagggaatgtgttcactttgttcccatgccatgaagagggtagggttaggtagtcacagacatctttttaaagccctgtctccttccaggatacacacaaatccgcttggtgaatggcaagaccccatgtgaaggaagagtggagctcaacattcttgggtcctgggggtccctctgcaactctcactgggacatggaagatgcccatgttttatgccagcagcttaaatgtggagttgccctttctatcccgggaggagcaccttttgggaaaggaagtgagcaggtctggaggcacatgtttcactgcactgggactgagaagcacatgggagattgttccgtcactgctctgggcgcatcactctgttcttcagggcaagtggcctctgtaatctgctcaggtaagagaataagggcagccagtgatgagccactcatgacggtgccttaagagtgggtgtacctaggagttcccattgtggctcagtggtaacaaactcgactggtatccatgagggtatgggtttgatccctggccttgctcaatgggttaaggatccagcattgctgtgagctgtggtataggttgcagactctgctcaggtcccatgttgctgtgattgtggtgtaggctgactgctgcagcttcaatttgacccctagcccgggaatttccataggccacacgtgcagcactaaggaaggaaaaaaagaaaaaaaaaaaaaaagagtgggtgtgcctatagtgaagaacagatgtaaaagggaagtgaaagggattcccccattctgagggattgtgagaagtgtgccagaatattaacttcatttgacttgttacagggaaagtaaacttgactttcacggacctcctagttacctggtgcttactatatgtcttctcagagtacctgattcattcccagcctggttgacccatccccctatctctatggctatgtttatccagagcacatctatctaacactccagctgatcttcctgacacagctgtggcaaccctggatcctttaaccaactgtgccaggctggagatcaaacctaagcctctgcagcaacccaagctgctgcagtcagatttttaaccccctgtgccactgtgggtatctccgatattttgtatcttctgtgactgagtggtttgctgtttgcagggaaccagagtcagacactatccccgtgcaattcatcatcctcggacccatcaagctctattatttcagaagaaaatggtgttgcctgcataggtgagaatcagtgaccaacctatgaaaatgatctcaatcctctgaaatgcattttattcatgttttatttcctctttgcagggagtggtcaacttcgcctggtcgatggaggtggtcgttgtgctgggagagtagaggtctatcatgagggctcctggggcaccatctgtgatgacagctgggacctgaatgatgcccatgtggtgtgcaaacagctgagctgtggatgggccattaatgccactggttctgctcattttggggaaggaacagggcccatttggctggatgagataaactgtaatggaaaagaatctcatatttggcaatgccactcacatggttgggggcggcacaattgcaggcataaggaggatgcaggagtcatctgctcgg

SEQ ID NO: 103 - DNA, 4615 bp, Sus scrofa
tatagatgacaaggctttgtgtctgataggggccagcgaactcagtaaagagggaagatgagaaagataatggcaagaatttatccctgaagtgtagttttgacaaaccagtcacaaagaggtctaagaaattttggtcacaaagttgttttgaatcccaggcattttatttgcaatgattgcatatgttctggaaaggacatctgaacctaagaaatagttcatttgcattgtgttatattttactaaggtctgagaaataatcttgagatgagaatgaactctacttcttcagagtctggaaggaataaattatgaaaatgtattaatgcttctttaaaccatattgtatatttatctattactaaacaaaaagaagtagctctatttatttatttatttatttatttatttatgtcttttgtctctttagggccacacctgtggcatatggaggttcccaggctagaggtccaattggagatgtagcagccagcctatgccagagccaccgcaacacgggatctgagccacgtctgtgacttacaccacagctcacagcaacgcctgatcctcaacccactgagcgaggccagggatcgaacccatgtcctcatggatgctagttgggttcgttaactgctgagccatgatgggaactccaaattaattatttcttatatttgttcttcatatattcatttctatagaaagaaataaatacagattcagttaatgatggcaggtaaaagcttaacttattaatcaaaggagttaatccaggcacaaaaattcaattcatggctctctgttaaaatttaggtataggtttagcaggaagaaaaggttagtagatgcagactattacatttagaatggatggacaatgaagtcctactatacagcacagggaactatatccaatctcttgggatagaatatgatggaagacaaaatcagaacaagagagtatatatatatgtgtgtgtgtgtgtgtgtgtgtgtgtgtgtgtgtgtgtgtgtgtgactgggtcaccctgcggcacagcagaaattggcagaacattgtaaatcaactatactttaataggaaaaatacttttaagggctaaatttccaatattctaaccatgtacacagagtaaatgtcataaggatgccagtctgtgtagagattgatgtgttactagcagattcatgaaataaaggctgaggatgtagtccccaagtcacttctgagtggaagaatttctcctttgtcctggactcaaatattttaggataaaggaaaaaagaagatatttatagaagggacttgttttcaagtacttgacaaaatttcaccattaaagagaaatttgtgggagttcccatcgtggctcagtggaaacaaatccaactaggaaccatgaggttgtgggtttgatccctggcctcactcagtgggttaaggatccggtgttgccgtgagctgtggtgtaggttgcagacacggttctgatcctgcgttgctgtggctgtggctgtggtgtaggccagcagcaaacagctctgattagacccctagcctggaaacctccatatgccacaggtgcagccctaaaaagacaaaaaaagagaaaagacaaaaaaaaaaaaaaaaaaaaaaaaaaaaaaaaaaaaaaaaaaaagaacccccagaggtatttatttgtttttgccttttttcactgactgttctttgtttgtttgtttgagactgatctagaagactagagattacaagaaatatggatttggctcactctaagaaactgctttcattccaaggtttgggtctatccaaaagtggaatagaatcatatgaatactagtttatgagtatttagtgagaggaatttcaagctcaaataatgattcagcaagattaaattaaggagggaattttccttgtggctgagtgggttaaggacccaatgttgtctctgtgaggatgtaggttccatcctgggctttgctcattaggttaaggatctggcattgctgcagctcagacccagtgctgccctggttgtggcttaggccaaagctgcagctccaattcaatctctggcctgggaacctccatgtgctacaaggtgcggccttaaaaggaaaaaaaaaaaattaaatcaaggactcaagagtctttcattatttgtgttgtggaagctatatttgttttaaagtcttagttgtgtttagaaagcaagatgttcttcaactcaaatttgggagggaacttgtttcatacatttttaatggataagtggcaaaattttcatgctgaggtgatctatagtgttgtaatgcagaatatagtcagatcttgaacattttaggaagttggtgagggccaattgtgtatctgtgccatgctgataagaatgtcaagggatcacaagaattcgtgttatttgacagcagtcatctttaaaaggcatttgagaaagtccaatttcaaatgcatttcctttctttaaaagataaattgaagaaaataagtctttatttcccaagtaaattgaattgcctctcagtctgttaaaagaaagaaggaaaatattggaatcatattctccctcaccgaaatgctatttttcagcccacaggaaacccaggctggttggaggggacattccctgctctggtcgtgttgaagtacaacatggagacacgtggggcaccgtctgtgattctgacttctctctggaggcggccagcgtgctgtgcagggaactacagtgcggcacagtgtggtttccctcctggggggagctcactttggagaaggaagtggacagatctgggctgaagaattccagtgtgaggggcacgagtcccacctttcactctgcccagtagcaccccgccctgacgggacatgtagccacagcagggacgtcggcgtagtctgctcaagtgagacccagggaatgtgttcactttgttcccatgccatgaagagggtagggttaggtagtcacagacatctttttaaagccctgtctccttccaggatacacacaaatccgcttggtgaatggcaagaccccatgtgaaggaagagtggagctcaacattcttgggtcctgggggtccctctgcaactctcactgggacatggaagatgcccatgttttatgccagcagcttaaatgtggagttgccctttctatcccgggaggagcaccttttgggaaaggaagtgagcaggtctggaggcacatgtttcactgcactgggactgagaagcacatgggagattgttccgtcactgctctgggcgcatcactctgttcttcagggcaagtggcctctgtaatctgctcaggtaagagaataagggcagccagtgatgagccactcatgacggtgccttaagagtgggtgtacctaggagttcccattgtggctcagtggtaacaaactcgactggtatccatgagggtatgggtttgatccctggccttgctcaatgggttaaggatccagcattgctgtgagctgtggtataggttgcagactctgctcaggtcccatgttgctgtgattgtggtgtaggctgactgctgcagcttcaatttgacccctagcccgggaatttccataggccacacgtgcagcactaaggaaggaaaaaaagaaaaaaaaaaaaaaagagtgggtgtgcctatagtgaagaacagatgtaaaagggaagtgaaagggattcccccattctgagggattgtgagaagtgtgccagaatattaacttcatttgacttgttacagggaaagtaaacttgactttcacggacctcctagttacctggtgcttactatatgtcttctcagagtacctgattcattcccagcctggttgacccatccccctatctctatggctatgtttatccagagcacatctatctaacactccagctgatcttcctgacacagctgtggcaaccctggatcctttaaccaactgtgccaggctggagatcaaacctaagcctctgcagcaacccaagctgctgcagtcagatttttaaccccctgtgccactgtgggtatctccgatattttgtatcttctgtgactgagtggtttgctgtttgcagggaaccagagtcagacactatccccgtgcaattcatcatcctcggacccatcaagctctattatttcagaagaaaatggtgttgcctgcataggtgagaatcagtgaccaacctatgaaaatgatctcaatcctctgaaatgcattttattcatgttttatttcctctttgcagggagtggtcaacttcgcctggtcgatggaggtggtcgttgtgctgggagagtagaggtctatcatgagggctcctggggcaccatctgtgatgacagctgggacctgaatgatgcccatgtggtgtgcaaacagctgagctgtggatgggccattaatgccactggttctgctcattttggggaaggaacagggcccatttggctggatgagataaactgtaatggaaaagaatctcatatttggcaatgccactcacatggttgggggcggcacaattgcaggcataaggaggatgcaggagtcatctgctcgg

SEQ ID NO: 104 - DNA, 4866 bp, Sus scrofa
tatagatgacaaggctttgtgtctgataggggccagcgaactcagtaaagagggaagatgagaaagataatggcaagaatttatccctgaagtgtagttttgacaaaccagtcacaaagaggtctaagaaattttggtcacaaagttgttttgaatcccaggcattttatttgcaatgattgcatatgttctggaaaggacatctgaacctaagaaatagttcatttgcattgtgttatattttactaaggtctgagaaataatcttgagatgagaatgaactctacttcttcagagtctggaaggaataaattatgaaaatgtattaatgcttctttaaaccatattgtatatttatctattactaaacaaaaagaagtagctctatttatttatttatttatttatttatttatgtcttttgtctctttagggccacacctgtggcatatggaggttcccaggctagaggtccaattggagatgtagcagccagcctatgccagagccaccgcaacacgggatctgagccacgtctgtgacttacaccacagctcacagcaacgcctgatcctcaacccactgagcgaggccagggatcgaacccatgtcctcatggatgctagttgggttcgttaactgctgagccatgatgggaactccaaattaattatttcttatatttgttcttcatatattcatttctatagaaagaaataaatacagattcagttaatgatggcaggtaaaagcttaacttattaatcaaaggagttaatccaggcacaaaaattcaattcatggctctctgttaaaatttaggtataggtttagcaggaagaaaaggttagtagatgcagactattacatttagaatggatggacaatgaagtcctactatacagcacagggaactatatccaatctcttgggatagaatatgatggaagacaaaatcagaacaagagagtatatatatatgtgtgtgtgtgtgtgtgtgtgtgtgtgtgtgtgtgtgtgtgtgtgactgggtcaccctgcggcacagcagaaattggcagaacattgtaaatcaactatactttaataggaaaaatacttttaagggctaaatttccaatattctaaccatgtacacagagtaaatgtcataaggatgccagtctgtgtagagattgatgtgttactagcagattcatgaaataaaggctgaggatgtagtccccaagtcacttctgagtggaagaatttctcctttgtcctggactcaaatattttaggataaaggaaaaaagaagatatttatagaagggacttgttttcaagtacttgacaaaatttcaccattaaagagaaatttgtgggagttcccatcgtggctcagtggaaacaaatccaactaggaaccatgaggttgtgggtttgatccctggcctcactcagtgggttaaggatccggtgttgccgtgagctgtggtgtaggttgcagacacggttctgatcctgcgttgctgtggctgtggctgtggtgtaggccagcagcaaacagctctgattagacccctagcctggaaacctccatatgccacaggtgcagccctaaaaagacaaaaaaagagaaaagacaaaaaaaaaaaaaaaaaaaaaaaaaaaaaaaaaaaaaaaaaaaagaacccccagaggtatttatttgtttttgccttttttcactgactgttctttgtttgtttgtttgagactgatctagaagactagagattacaagaaatatggatttggctcactctaagaaactgctttcattccaaggtttgggtctatccaaaagtggaatagaatcatatgaatactagtttatgagtatttagtgagaggaatttcaagctcaaataatgattcagcaagattaaattaaggagggaattttccttgtggctgagtgggttaaggacccaatgttgtctctgtgaggatgtaggttccatcctgggctttgctcattaggttaaggatctggcattgctgcagctcagacccagtgctgccctggttgtggcttaggccaaagctgcagctccaattcaatctctggcctgggaacctccatgtgctacaaggtgcggccttaaaaggaaaaaaaaaaaattaaatcaaggactcaagagtctttcattatttgtgttgtggaagctatatttgttttaaagtcttagttgtgtttagaaagcaagatgttcttcaactcaaatttgggagggaacttgtttcatacatttttaatggataagtggcaaaattttcatgctgaggtgatctatagtgttgtaatgcagaatatagtcagatcttgaacattttaggaagttggtgagggccaattgtgtatctgtgccatgctgataagaatgtcaagggatcacaagaattcgtgttatttgacagcagtcatctttaaaaggcatttgagaaagtccaatttcaaatgcatttcctttctttaaaagataaattgaagaaaataagtctttatttcccaagtaaattgaattgcctctcagtctgttaaaagaaactcttaccttgatgattgcgctcttaacctggcaaagattgtctttaaaatctgagctccatgtcttctgctttatttctggtgtgcctttgactccagattacagtaaatggaggactgagtatagggctaaaaagtagagagaatggatgcatattatctgtggtctccaatgtgatgaatgaagtaggcaaatactcaaaggaaagagaaagcatgctccaagaattatgggttccagaaggcaaagtcccagaattgtctccagggaaggacagggaggtctagaatcggctaagcccactgtaggcagaaaaaccaagaggcatgaatggcttccctttctcacttttcactctctggcttactcctatcatgaaggaaaatattggaatcatattctccctcaccgaaatgctatttttcagcccacaggaaacccaggctggttctgtggtttccctcctggggggagctcactttggagaaggaagtggacagatctgggctgaagaattccagtgtgaggggcacgagtcccacctttcactctgcccagtagcaccccgccctgacgggacatgtagccacagcagggacgtcggcgtagtctgctcaagtgagacccagggaatgtgttcactttgttcccatgccatgaagagggtagggttaggtagtcacagacatctttttaaagccctgtctccttccaggatacacacaaatccgcttggtgaatggcaagaccccatgtgaaggaagagtggagctcaacattcttgggtcctgggggtccctctgcaactctcactgggacatggaagatgcccatgttttatgccagcagcttaaatgtggagttgccctttctatcccgggaggagcaccttttgggaaaggaagtgagcaggtctggaggcacatgtttcactgcactgggactgagaagcacatgggagattgttccgtcactgctctgggcgcatcactctgttcttcagggcaagtggcctctgtaatctgctcaggtaagagaataagggcagccagtgatgagccactcatgacggtgccttaagagtgggtgtacctaggagttcccattgtggctcagtggtaacaaactcgactggtatccatgagggtatgggtttgatccctggccttgctcaatgggttaaggatccagcattgctgtgagctgtggtataggttgcagactctgctcaggtcccatgttgctgtgattgtggtgtaggctgactgctgcagcttcaatttgacccctagcccgggaatttccataggccacacgtgcagcactaaggaaggaaaaaaagaaaaaaaaaaaaaaagagtgggtgtgcctatagtgaagaacagatgtaaaagggaagtgaaagggattcccccattctgagggattgtgagaagtgtgccagaatattaacttcatttgacttgttacagggaaagtaaacttgactttcacggacctcctagttacctggtgcttactatatgtcttctcagagtacctgattcattcccagcctggttgacccatccccctatctctatggctatgtttatccagagcacatctatctaacactccagctgatcttcctgacacagctgtggcaaccctggatcctttaaccaactgtgccaggctggagatcaaacctaagcctctgcagcaacccaagctgctgcagtcagatttttaaccccctgtgccactgtgggtatctccgatattttgtatcttctgtgactgagtggtttgctgtttgcagggaaccagagtcagacactatccccgtgcaattcatcatcctcggacccatcaagctctattatttcagaagaaaatggtgttgcctgcataggtgagaatcagtgaccaacctatgaaaatgatctcaatcctctgaaatgcattttattcatgttttatttcctctttgcagggagtggtcaacttcgcctggtcgatggaggtggtcgttgtgctgggagagtagaggtctatcatgagggctcctggggcaccatctgtgatgacagctgggacctgaatgatgcccatgtggtgtgcaaacagctgagctgtggatgggccattaatgccactggttctgctcattttggggaaggaacagggcccatttggctggatgagataaactgtaatggaaaagaatctcatatttggcaatgccactcacatggttgggggcggcacaattgcaggcataaggaggatgcaggagtcatctgctcgg

SEQ ID NO: 105 - DNA, 4867 bp, Sus scrofa
tatagatgacaaggctttgtgtctgataggggccagcgaactcagtaaagagggaagatgagaaagataatggcaagaatttatccctgaagtgtagttttgacaaaccagtcacaaagaggtctaagaaattttggtcacaaagttgttttgaatcccaggcattttatttgcaatgattgcatatgttctggaaaggacatctgaacctaagaaatagttcatttgcattgtgttatattttactaaggtctgagaaataatcttgagatgagaatgaactctacttcttcagagtctggaaggaataaattatgaaaatgtattaatgcttctttaaaccatattgtatatttatctattactaaacaaaaagaagtagctctatttatttatttatttatttatttatttatgtcttttgtctctttagggccacacctgtggcatatggaggttcccaggctagaggtccaattggagatgtagcagccagcctatgccagagccaccgcaacacgggatctgagccacgtctgtgacttacaccacagctcacagcaacgcctgatcctcaacccactgagcgaggccagggatcgaacccatgtcctcatggatgctagttgggttcgttaactgctgagccatgatgggaactccaaattaattatttcttatatttgttcttcatatattcatttctatagaaagaaataaatacagattcagttaatgatggcaggtaaaagcttaacttattaatcaaaggagttaatccaggcacaaaaattcaattcatggctctctgttaaaatttaggtataggtttagcaggaagaaaaggttagtagatgcagactattacatttagaatggatggacaatgaagtcctactatacagcacagggaactatatccaatctcttgggatagaatatgatggaagacaaaatcagaacaagagagtatatatatatgtgtgtgtgtgtgtgtgtgtgtgtgtgtgtgtgtgtgtgtgtgtgactgggtcaccctgcggcacagcagaaattggcagaacattgtaaatcaactatactttaataggaaaaatacttttaagggctaaatttccaatattctaaccatgtacacagagtaaatgtcataaggatgccagtctgtgtagagattgatgtgttactagcagattcatgaaataaaggctgaggatgtagtccccaagtcacttctgagtggaagaatttctcctttgtcctggactcaaatattttaggataaaggaaaaaagaagatatttatagaagggacttgttttcaagtacttgacaaaatttcaccattaaagagaaatttgtgggagttcccatcgtggctcagtggaaacaaatccaactaggaaccatgaggttgtgggtttgatccctggcctcactcagtgggttaaggatccggtgttgccgtgagctgtggtgtaggttgcagacacggttctgatcctgcgttgctgtggctgtggctgtggtgtaggccagcagcaaacagctctgattagacccctagcctggaaacctccatatgccacaggtgcagccctaaaaagacaaaaaaagagaaaagacaaaaaaaaaaaaaaaaaaaaaaaaaaaaaaaaaaaaaaaaaaaagaacccccagaggtatttatttgtttttgccttttttcactgactgttctttgtttgtttgtttgagactgatctagaagactagagattacaagaaatatggatttggctcactctaagaaactgctttcattccaaggtttgggtctatccaaaagtggaatagaatcatatgaatactagtttatgagtatttagtgagaggaatttcaagctcaaataatgattcagcaagattaaattaaggagggaattttccttgtggctgagtgggttaaggacccaatgttgtctctgtgaggatgtaggttccatcctgggctttgctcattaggttaaggatctggcattgctgcagctcagacccagtgctgccctggttgtggcttaggccaaagctgcagctccaattcaatctctggcctgggaacctccatgtgctacaaggtgcggccttaaaaggaaaaaaaaaaaattaaatcaaggactcaagagtctttcattatttgtgttgtggaagctatatttgttttaaagtcttagttgtgtttagaaagcaagatgttcttcaactcaaatttgggagggaacttgtttcatacatttttaatggataagtggcaaaattttcatgctgaggtgatctatagtgttgtaatgcagaatatagtcagatcttgaacattttaggaagttggtgagggccaattgtgtatctgtgccatgctgataagaatgtcaagggatcacaagaattcgtgttatttgacagcagtcatctttaaaaggcatttgagaaagtccaatttcaaatgcatttcctttctttaaaagataaattgaagaaaataagtctttatttcccaagtaaattgaattgcctctcagtctgttaaaagaaactcttaccttgatgattgcgctcttaacctggcaaagattgtctttaaaatctgagctccatgtcttctgctttatttctggtgtgcctttgactccagattacagtaaatggaggactgagtatagggctaaaaagtagagagaatggatgcatattatctgtggtctccaatgtgatgaatgaagtaggcaaatactcaaaggaaagagaaagcatgctccaagaattatgggttccagaaggcaaagtcccagaattgtctccagggaaggacagggaggtctagaatcggctaagcccactgtaggcagaaaaaccaagaggcatgaatggcttccctttctcacttttcactctctggcttactcctatcatgaaggaaaatattggaatcatattctccctcaccgaaatgctatttttcagcccacaggaaacccaggctggttactgtggtttccctcctggggggagctcactttggagaaggaagtggacagatctgggctgaagaattccagtgtgaggggcacgagtcccacctttcactctgcccagtagcaccccgccctgacgggacatgtagccacagcagggacgtcggcgtagtctgctcaagtgagacccagggaatgtgttcactttgttcccatgccatgaagagggtagggttaggtagtcacagacatctttttaaagccctgtctccttccaggatacacacaaatccgcttggtgaatggcaagaccccatgtgaaggaagagtggagctcaacattcttgggtcctgggggtccctctgcaactctcactgggacatggaagatgcccatgttttatgccagcagcttaaatgtggagttgccctttctatcccgggaggagcaccttttgggaaaggaagtgagcaggtctggaggcacatgtttcactgcactgggactgagaagcacatgggagattgttccgtcactgctctgggcgcatcactctgttcttcagggcaagtggcctctgtaatctgctcaggtaagagaataagggcagccagtgatgagccactcatgacggtgccttaagagtgggtgtacctaggagttcccattgtggctcagtggtaacaaactcgactggtatccatgagggtatgggtttgatccctggccttgctcaatgggttaaggatccagcattgctgtgagctgtggtataggttgcagactctgctcaggtcccatgttgctgtgattgtggtgtaggctgactgctgcagcttcaatttgacccctagcccgggaatttccataggccacacgtgcagcactaaggaaggaaaaaaagaaaaaaaaaaaaaaagagtgggtgtgcctatagtgaagaacagatgtaaaagggaagtgaaagggattcccccattctgagggattgtgagaagtgtgccagaatattaacttcatttgacttgttacagggaaagtaaacttgactttcacggacctcctagttacctggtgcttactatatgtcttctcagagtacctgattcattcccagcctggttgacccatccccctatctctatggctatgtttatccagagcacatctatctaacactccagctgatcttcctgacacagctgtggcaaccctggatcctttaaccaactgtgccaggctggagatcaaacctaagcctctgcagcaacccaagctgctgcagtcagatttttaaccccctgtgccactgtgggtatctccgatattttgtatcttctgtgactgagtggtttgctgtttgcagggaaccagagtcagacactatccccgtgcaattcatcatcctcggacccatcaagctctattatttcagaagaaaatggtgttgcctgcataggtgagaatcagtgaccaacctatgaaaatgatctcaatcctctgaaatgcattttattcatgttttatttcctctttgcagggagtggtcaacttcgcctggtcgatggaggtggtcgttgtgctgggagagtagaggtctatcatgagggctcctggggcaccatctgtgatgacagctgggacctgaatgatgcccatgtggtgtgcaaacagctgagctgtggatgggccattaatgccactggttctgctcattttggggaaggaacagggcccatttggctggatgagataaactgtaatggaaaagaatctcatatttggcaatgccactcacatggttgggggcggcacaattgcaggcataaggaggatgcaggagtcatctgctcgg

SEQ ID NO: 106 - DNA, 4991 bp, Sus scrofa
tatagatgacaaggctttgtgtctgataggggccagcgaactcagtaaagagggaagatgagaaagataatggcaagaatttatccctgaagtgtagttttgacaaaccagtcacaaagaggtctaagaaattttggtcacaaagttgttttgaatcccaggcattttatttgcaatgattgcatatgttctggaaaggacatctgaacctaagaaatagttcatttgcattgtgttatattttactaaggtctgagaaataatcttgagatgagaatgaactctacttcttcagagtctggaaggaataaattatgaaaatgtattaatgcttctttaaaccatattgtatatttatctattactaaacaaaaagaagtagctctatttatttatttatttatttatttatttatgtcttttgtctctttagggccacacctgtggcatatggaggttcccaggctagaggtccaattggagatgtagcagccagcctatgccagagccaccgcaacacgggatctgagccacgtctgtgacttacaccacagctcacagcaacgcctgatcctcaacccactgagcgaggccagggatcgaacccatgtcctcatggatgctagttgggttcgttaactgctgagccatgatgggaactccaaattaattatttcttatatttgttcttcatatattcatttctatagaaagaaataaatacagattcagttaatgatggcaggtaaaagcttaacttattaatcaaaggagttaatccaggcacaaaaattcaattcatggctctctgttaaaatttaggtataggtttagcaggaagaaaaggttagtagatgcagactattacatttagaatggatggacaatgaagtcctactatacagcacagggaactatatccaatctcttgggatagaatatgatggaagacaaaatcagaacaagagagtatatatatatgtgtgtgtgtgtgtgtgtgtgtgtgtgtgtgtgtgtgtgtgtgtgactgggtcaccctgcggcacagcagaaattggcagaacattgtaaatcaactatactttaataggaaaaatacttttaagggctaaatttccaatattctaaccatgtacacagagtaaatgtcataaggatgccagtctgtgtagagattgatgtgttactagcagattcatgaaataaaggctgaggatgtagtccccaagtcacttctgagtggaagaatttctcctttgtcctggactcaaatattttaggataaaggaaaaaagaagatatttatagaagggacttgttttcaagtacttgacaaaatttcaccattaaagagaaatttgtgggagttcccatcgtggctcagtggaaacaaatccaactaggaaccatgaggttgtgggtttgatccctggcctcactcagtgggttaaggatccggtgttgccgtgagctgtggtgtaggttgcagacacggttctgatcctgcgttgctgtggctgtggctgtggtgtaggccagcagcaaacagctctgattagacccctagcctggaaacctccatatgccacaggtgcagccctaaaaagacaaaaaaagagaaaagacaaaaaaaaaaaaaaaaaaaaaaaaaaaaaaaaaaaaaaaaaaaagaacccccagaggtatttatttgtttttgccttttttcactgactgttctttgtttgtttgtttgagactgatctagaagactagagattacaagaaatatggatttggctcactctaagaaactgctttcattccaaggtttgggtctatccaaaagtggaatagaatcatatgaatactagtttatgagtatttagtgagaggaatttcaagctcaaataatgattcagcaagattaaattaaggagggaattttccttgtggctgagtgggttaaggacccaatgttgtctctgtgaggatgtaggttccatcctgggctttgctcattaggttaaggatctggcattgctgcagctcagacccagtgctgccctggttgtggcttaggccaaagctgcagctccaattcaatctctggcctgggaacctccatgtgctacaaggtgcggccttaaaaggaaaaaaaaaaaattaaatcaaggactcaagagtctttcattatttgtgttgtggaagctatatttgttttaaagtcttagttgtgtttagaaagcaagatgttcttcaactcaaatttgggagggaacttgtttcatacatttttaatggataagtggcaaaattttcatgctgaggtgatctatagtgttgtaatgcagaatatagtcagatcttgaacattttaggaagttggtgagggccaattgtgtatctgtgccatgctgataagaatgtcaagggatcacaagaattcgtgttatttgacagcagtcatctttaaaaggcatttgagaaagtccaatttcaaatgcatttcctttctttaaaagataaattgaagaaaataagtctttatttcccaagtaaattgaattgcctctcagtctgttaaaagaaactcttaccttgatgattgcgctcttaacctggcaaagattgtctttaaaatctgagctccatgtcttctgctttatttctggtgtgcctttgactccagattacagtaaatggaggactgagtatagggctaaaaagtagagagaatggatgcatattatctgtggtctccaatgtgatgaatgaagtaggcaaatactcaaaggaaagagaaagcatgctccaagaattatgggttccagaaggcaaagtcccagaattgtctccagggaaggacagggaggtctagaatcggctaagcccactgtaggcagaaaaaccaagaggcatgaatggcttccctttctcacttttcactctctggcttactcctatcatgaaggaaaatattggaatcatattctccctcaccgaaatgctatttttcagcccacaggaaacccaggctggttggaggggacattccctgctctggtcgtgttgaagtacaacatggagacacgtggggcaccgtctgtgattctgacttctctctggaggcggccagcgtgctgtgcagggaactacagtgcggcaactgtggtttccctcctggggggagctcactttggagaaggaagtggacagatctgggctgaagaattccagtgtgaggggcacgagtcccacctttcactctgcccagtagcaccccgccctgacgggacatgtagccacagcagggacgtcggcgtagtctgctcaagtgagacccagggaatgtgttcactttgttcccatgccatgaagagggtagggttaggtagtcacagacatctttttaaagccctgtctccttccaggatacacacaaatccgcttggtgaatggcaagaccccatgtgaaggaagagtggagctcaacattcttgggtcctgggggtccctctgcaactctcactgggacatggaagatgcccatgttttatgccagcagcttaaatgtggagttgccctttctatcccgggaggagcaccttttgggaaaggaagtgagcaggtctggaggcacatgtttcactgcactgggactgagaagcacatgggagattgttccgtcactgctctgggcgcatcactctgttcttcagggcaagtggcctctgtaatctgctcaggtaagagaataagggcagccagtgatgagccactcatgacggtgccttaagagtgggtgtacctaggagttcccattgtggctcagtggtaacaaactcgactggtatccatgagggtatgggtttgatccctggccttgctcaatgggttaaggatccagcattgctgtgagctgtggtataggttgcagactctgctcaggtcccatgttgctgtgattgtggtgtaggctgactgctgcagcttcaatttgacccctagcccgggaatttccataggccacacgtgcagcactaaggaaggaaaaaaagaaaaaaaaaaaaaaagagtgggtgtgcctatagtgaagaacagatgtaaaagggaagtgaaagggattcccccattctgagggattgtgagaagtgtgccagaatattaacttcatttgacttgttacagggaaagtaaacttgactttcacggacctcctagttacctggtgcttactatatgtcttctcagagtacctgattcattcccagcctggttgacccatccccctatctctatggctatgtttatccagagcacatctatctaacactccagctgatcttcctgacacagctgtggcaaccctggatcctttaaccaactgtgccaggctggagatcaaacctaagcctctgcagcaacccaagctgctgcagtcagatttttaaccccctgtgccactgtgggtatctccgatattttgtatcttctgtgactgagtggtttgctgtttgcagggaaccagagtcagacactatccccgtgcaattcatcatcctcggacccatcaagctctattatttcagaagaaaatggtgttgcctgcataggtgagaatcagtgaccaacctatgaaaatgatctcaatcctctgaaatgcattttattcatgttttatttcctctttgcagggagtggtcaacttcgcctggtcgatggaggtggtcgttgtgctgggagagtagaggtctatcatgagggctcctggggcaccatctgtgatgacagctgggacctgaatgatgcccatgtggtgtgcaaacagctgagctgtggatgggccattaatgccactggttctgctcattttggggaaggaacagggcccatttggctggatgagataaactgtaatggaaaagaatctcatatttggcaatgccactcacatggttgggggcggcacaattgcaggcataaggaggatgcaggagtcatctgctcgg

SEQ ID NO: 107 - DNA, 4860 bp, Sus scrofa
tatagatgacaaggctttgtgtctgataggggccagcgaactcagtaaagagggaagatgagaaagataatggcaagaatttatccctgaagtgtagttttgacaaaccagtcacaaagaggtctaagaaattttggtcacaaagttgttttgaatcccaggcattttatttgcaatgattgcatatgttctggaaaggacatctgaacctaagaaatagttcatttgcattgtgttatattttactaaggtctgagaaataatcttgagatgagaatgaactctacttcttcagagtctggaaggaataaattatgaaaatgtattaatgcttctttaaaccatattgtatatttatctattactaaacaaaaagaagtagctctatttatttatttatttatttatttatttatgtcttttgtctctttagggccacacctgtggcatatggaggttcccaggctagaggtccaattggagatgtagcagccagcctatgccagagccaccgcaacacgggatctgagccacgtctgtgacttacaccacagctcacagcaacgcctgatcctcaacccactgagcgaggccagggatcgaacccatgtcctcatggatgctagttgggttcgttaactgctgagccatgatgggaactccaaattaattatttcttatatttgttcttcatatattcatttctatagaaagaaataaatacagattcagttaatgatggcaggtaaaagcttaacttattaatcaaaggagttaatccaggcacaaaaattcaattcatggctctctgttaaaatttaggtataggtttagcaggaagaaaaggttagtagatgcagactattacatttagaatggatggacaatgaagtcctactatacagcacagggaactatatccaatctcttgggatagaatatgatggaagacaaaatcagaacaagagagtatatatatatgtgtgtgtgtgtgtgtgtgtgtgtgtgtgtgtgtgtgtgtgtgtgactgggtcaccctgcggcacagcagaaattggcagaacattgtaaatcaactatactttaataggaaaaatacttttaagggctaaatttccaatattctaaccatgtacacagagtaaatgtcataaggatgccagtctgtgtagagattgatgtgttactagcagattcatgaaataaaggctgaggatgtagtccccaagtcacttctgagtggaagaatttctcctttgtcctggactcaaatattttaggataaaggaaaaaagaagatatttatagaagggacttgttttcaagtacttgacaaaatttcaccattaaagagaaatttgtgggagttcccatcgtggctcagtggaaacaaatccaactaggaaccatgaggttgtgggtttgatccctggcctcactcagtgggttaaggatccggtgttgccgtgagctgtggtgtaggttgcagacacggttctgatcctgcgttgctgtggctgtggctgtggtgtaggccagcagcaaacagctctgattagacccctagcctggaaacctccatatgccacaggtgcagccctaaaaagacaaaaaaagagaaaagacaaaaaaaaaaaaaaaaaaaaaaaaaaaaaaaaaaaaaaaaaaaagaacccccagaggtatttatttgtttttgccttttttcactgactgttctttgtttgtttgtttgagactgatctagaagactagagattacaagaaatatggatttggctcactctaagaaactgctttcattccaaggtttgggtctatccaaaagtggaatagaatcatatgaatactagtttatgagtatttagtgagaggaatttcaagctcaaataatgattcagcaagattaaattaaggagggaattttccttgtggctgagtgggttaaggacccaatgttgtctctgtgaggatgtaggttccatcctgggctttgctcattaggttaaggatctggcattgctgcagctcagacccagtgctgccctggttgtggcttaggccaaagctgcagctccaattcaatctctggcctgggaacctccatgtgctacaaggtgcggccttaaaaggaaaaaaaaaaaattaaatcaaggactcaagagtctttcattatttgtgttgtggaagctatatttgttttaaagtcttagttgtgtttagaaagcaagatgttcttcaactcaaatttgggagggaacttgtttcatacatttttaatggataagtggcaaaattttcatgctgaggtgatctatagtgttgtaatgcagaatatagtcagatcttgaacattttaggaagttggtgagggccaattgtgtatctgtgccatgctgataagaatgtcaagggatcacaagaattcgtgttatttgacagcagtcatctttaaaaggcatttgagaaagtccaatttcaaatgcatttcctttctttaaaagataaattgaagaaaataagtctttatttcccaagtaaattgaattgcctctcagtctgttaaaagaaactcttaccttgatgattgcgctcttaacctggcaaagattgtctttaaaatctgagctccatgtcttctgctttatttctggtgtgcctttgactccagattacagtaaatggaggactgagtatagggctaaaaagtagagagaatggatgcatattatctgtggtctccaatgtgatgaatgaagtaggcaaatactcaaaggaaagagaaagcatgctccaagaattatgggttccagaaggcaaagtcccagaattgtctccagggaaggacagggaggtctagaatcggctaagcccactgtaggcagaaaaaccaagaggcatgaatggcttccctttctcacttttcactctctggcttactcctatcatgaaggaaaatattggaatcatattctccctcaccgaaatgctatttttcagcccacaggaaacccaggctggttggagggtcctggggggagctcactttggagaaggaagtggacagatctgggctgaagaattccagtgtgaggggcacgagtcccacctttcactctgcccagtagcaccccgccctgacgggacatgtagccacagcagggacgtcggcgtagtctgctcaagtgagacccagggaatgtgttcactttgttcccatgccatgaagagggtagggttaggtagtcacagacatctttttaaagccctgtctccttccaggatacacacaaatccgcttggtgaatggcaagaccccatgtgaaggaagagtggagctcaacattcttgggtcctgggggtccctctgcaactctcactgggacatggaagatgcccatgttttatgccagcagcttaaatgtggagttgccctttctatcccgggaggagcaccttttgggaaaggaagtgagcaggtctggaggcacatgtttcactgcactgggactgagaagcacatgggagattgttccgtcactgctctgggcgcatcactctgttcttcagggcaagtggcctctgtaatctgctcaggtaagagaataagggcagccagtgatgagccactcatgacggtgccttaagagtgggtgtacctaggagttcccattgtggctcagtggtaacaaactcgactggtatccatgagggtatgggtttgatccctggccttgctcaatgggttaaggatccagcattgctgtgagctgtggtataggttgcagactctgctcaggtcccatgttgctgtgattgtggtgtaggctgactgctgcagcttcaatttgacccctagcccgggaatttccataggccacacgtgcagcactaaggaaggaaaaaaagaaaaaaaaaaaaaaagagtgggtgtgcctatagtgaagaacagatgtaaaagggaagtgaaagggattcccccattctgagggattgtgagaagtgtgccagaatattaacttcatttgacttgttacagggaaagtaaacttgactttcacggacctcctagttacctggtgcttactatatgtcttctcagagtacctgattcattcccagcctggttgacccatccccctatctctatggctatgtttatccagagcacatctatctaacactccagctgatcttcctgacacagctgtggcaaccctggatcctttaaccaactgtgccaggctggagatcaaacctaagcctctgcagcaacccaagctgctgcagtcagatttttaaccccctgtgccactgtgggtatctccgatattttgtatcttctgtgactgagtggtttgctgtttgcagggaaccagagtcagacactatccccgtgcaattcatcatcctcggacccatcaagctctattatttcagaagaaaatggtgttgcctgcataggtgagaatcagtgaccaacctatgaaaatgatctcaatcctctgaaatgcattttattcatgttttatttcctctttgcagggagtggtcaacttcgcctggtcgatggaggtggtcgttgtgctgggagagtagaggtctatcatgagggctcctggggcaccatctgtgatgacagctgggacctgaatgatgcccatgtggtgtgcaaacagctgagctgtggatgggccattaatgccactggttctgctcattttggggaaggaacagggcccatttggctggatgagataaactgtaatggaaaagaatctcatatttggcaatgccactcacatggttgggggcggcacaattgcaggcataaggaggatgcaggagtcatctgctcgg

SEQ ID NO: 108 - DNA, 4858 bp, Sus scrofa
tatagatgacaaggctttgtgtctgataggggccagcgaactcagtaaagagggaagatgagaaagataatggcaagaatttatccctgaagtgtagttttgacaaaccagtcacaaagaggtctaagaaattttggtcacaaagttgttttgaatcccaggcattttatttgcaatgattgcatatgttctggaaaggacatctgaacctaagaaatagttcatttgcattgtgttatattttactaaggtctgagaaataatcttgagatgagaatgaactctacttcttcagagtctggaaggaataaattatgaaaatgtattaatgcttctttaaaccatattgtatatttatctattactaaacaaaaagaagtagctctatttatttatttatttatttatttatttatgtcttttgtctctttagggccacacctgtggcatatggaggttcccaggctagaggtccaattggagatgtagcagccagcctatgccagagccaccgcaacacgggatctgagccacgtctgtgacttacaccacagctcacagcaacgcctgatcctcaacccactgagcgaggccagggatcgaacccatgtcctcatggatgctagttgggttcgttaactgctgagccatgatgggaactccaaattaattatttcttatatttgttcttcatatattcatttctatagaaagaaataaatacagattcagttaatgatggcaggtaaaagcttaacttattaatcaaaggagttaatccaggcacaaaaattcaattcatggctctctgttaaaatttaggtataggtttagcaggaagaaaaggttagtagatgcagactattacatttagaatggatggacaatgaagtcctactatacagcacagggaactatatccaatctcttgggatagaatatgatggaagacaaaatcagaacaagagagtatatatatatgtgtgtgtgtgtgtgtgtgtgtgtgtgtgtgtgtgtgtgtgtgtgactgggtcaccctgcggcacagcagaaattggcagaacattgtaaatcaactatactttaataggaaaaatacttttaagggctaaatttccaatattctaaccatgtacacagagtaaatgtcataaggatgccagtctgtgtagagattgatgtgttactagcagattcatgaaataaaggctgaggatgtagtccccaagtcacttctgagtggaagaatttctcctttgtcctggactcaaatattttaggataaaggaaaaaagaagatatttatagaagggacttgttttcaagtacttgacaaaatttcaccattaaagagaaatttgtgggagttcccatcgtggctcagtggaaacaaatccaactaggaaccatgaggttgtgggtttgatccctggcctcactcagtgggttaaggatccggtgttgccgtgagctgtggtgtaggttgcagacacggttctgatcctgcgttgctgtggctgtggctgtggtgtaggccagcagcaaacagctctgattagacccctagcctggaaacctccatatgccacaggtgcagccctaaaaagacaaaaaaagagaaaagacaaaaaaaaaaaaaaaaaaaaaaaaaaaaaaaaaaaaaaaaaaaagaacccccagaggtatttatttgtttttgccttttttcactgactgttctttgtttgtttgtttgagactgatctagaagactagagattacaagaaatatggatttggctcactctaagaaactgctttcattccaaggtttgggtctatccaaaagtggaatagaatcatatgaatactagtttatgagtatttagtgagaggaatttcaagctcaaataatgattcagcaagattaaattaaggagggaattttccttgtggctgagtgggttaaggacccaatgttgtctctgtgaggatgtaggttccatcctgggctttgctcattaggttaaggatctggcattgctgcagctcagacccagtgctgccctggttgtggcttaggccaaagctgcagctccaattcaatctctggcctgggaacctccatgtgctacaaggtgcggccttaaaaggaaaaaaaaaaaattaaatcaaggactcaagagtctttcattatttgtgttgtggaagctatatttgttttaaagtcttagttgtgtttagaaagcaagatgttcttcaactcaaatttgggagggaacttgtttcatacatttttaatggataagtggcaaaattttcatgctgaggtgatctatagtgttgtaatgcagaatatagtcagatcttgaacattttaggaagttggtgagggccaattgtgtatctgtgccatgctgataagaatgtcaagggatcacaagaattcgtgttatttgacagcagtcatctttaaaaggcatttgagaaagtccaatttcaaatgcatttcctttctttaaaagataaattgaagaaaataagtctttatttcccaagtaaattgaattgcctctcagtctgttaaaagaaactcttaccttgatgattgcgctcttaacctggcaaagattgtctttaaaatctgagctccatgtcttctgctttatttctggtgtgcctttgactccagattacagtaaatggaggactgagtatagggctaaaaagtagagagaatggatgcatattatctgtggtctccaatgtgatgaatgaagtaggcaaatactcaaaggaaagagaaagcatgctccaagaattatgggttccagaaggcaaagtcccagaattgtctccagggaaggacagggaggtctagaatcggctaagcccactgtaggcagaaaaaccaagaggcatgaatggcttccctttctcacttttcactctctggcttactcctatcatgaaggaaaatattggaatcatattctccctcaccgaaatgctatttttcagcccacaggaaacccaggctggttggagggctggggggagctcactttggagaaggaagtggacagatctgggctgaagaattccagtgtgaggggcacgagtcccacctttcactctgcccagtagcaccccgccctgacgggacatgtagccacagcagggacgtcggcgtagtctgctcaagtgagacccagggaatgtgttcactttgttcccatgccatgaagagggtagggttaggtagtcacagacatctttttaaagccctgtctccttccaggatacacacaaatccgcttggtgaatggcaagaccccatgtgaaggaagagtggagctcaacattcttgggtcctgggggtccctctgcaactctcactgggacatggaagatgcccatgttttatgccagcagcttaaatgtggagttgccctttctatcccgggaggagcaccttttgggaaaggaagtgagcaggtctggaggcacatgtttcactgcactgggactgagaagcacatgggagattgttccgtcactgctctgggcgcatcactctgttcttcagggcaagtggcctctgtaatctgctcaggtaagagaataagggcagccagtgatgagccactcatgacggtgccttaagagtgggtgtacctaggagttcccattgtggctcagtggtaacaaactcgactggtatccatgagggtatgggtttgatccctggccttgctcaatgggttaaggatccagcattgctgtgagctgtggtataggttgcagactctgctcaggtcccatgttgctgtgattgtggtgtaggctgactgctgcagcttcaatttgacccctagcccgggaatttccataggccacacgtgcagcactaaggaaggaaaaaaagaaaaaaaaaaaaaaagagtgggtgtgcctatagtgaagaacagatgtaaaagggaagtgaaagggattcccccattctgagggattgtgagaagtgtgccagaatattaacttcatttgacttgttacagggaaagtaaacttgactttcacggacctcctagttacctggtgcttactatatgtcttctcagagtacctgattcattcccagcctggttgacccatccccctatctctatggctatgtttatccagagcacatctatctaacactccagctgatcttcctgacacagctgtggcaaccctggatcctttaaccaactgtgccaggctggagatcaaacctaagcctctgcagcaacccaagctgctgcagtcagatttttaaccccctgtgccactgtgggtatctccgatattttgtatcttctgtgactgagtggtttgctgtttgcagggaaccagagtcagacactatccccgtgcaattcatcatcctcggacccatcaagctctattatttcagaagaaaatggtgttgcctgcataggtgagaatcagtgaccaacctatgaaaatgatctcaatcctctgaaatgcattttattcatgttttatttcctctttgcagggagtggtcaacttcgcctggtcgatggaggtggtcgttgtgctgggagagtagaggtctatcatgagggctcctggggcaccatctgtgatgacagctgggacctgaatgatgcccatgtggtgtgcaaacagctgagctgtggatgggccattaatgccactggttctgctcattttggggaaggaacagggcccatttggctggatgagataaactgtaatggaaaagaatctcatatttggcaatgccactcacatggttgggggcggcacaattgcaggcataaggaggatgcaggagtcatctgctcgg

SEQ ID NO: 109 - DNA, 3523 bp, Sus scrofa
tatagatgacaaggctttgtgtctgataggggccagcgaactcagtaaagagggaagatgagaaagataatggcaagaatttatccctgaagtgtagttttgacaaaccagtcacaaagaggtctaagaaattttggtcacaaagttgttttgaatcccaggcattttatttgcaatgattgcatatgttctggaaaggacatctgaacctaagaaatagttcatttgcattgtgttatattttactaaggtctgagaaataatcttgagatgagaatgaactctacttcttcagagtctggaaggaataaattatgaaaatgtattaatgcttctttaaaccatattgtatatttatctattactaaacaaaaagaagtagctctatttatttatttatttatttatttatttatgtcttttgtctctttagggccacacctgtggcatatggaggttcccaggctagaggtccaattggagatgtagcagccagcctatgccagagccaccgcaacacgggatctgagccacgtctgtgacttacaccacagctcacagcaacgcctgatcctcaacccactgagcgaggccagggatcgaacccatgtcctcatggatgctagttgggttcgttaactgctgagccatgatgggaactccaaattaattatttcttatatttgttcttcatatattcatttctatagaaagaaataaatacagattcagttaatgatggcaggtaaaagcttaacttattaatcaaaggagttaatccaggcacaaaaattcaattcatggctctctgttaaaatttaggtataggtttagcaggaagaaaaggttagtagatgcagactattacatttagaatggatggacaatgaagtcctactatacagcacagggaactatatccaatctcttgggatagaatatgatggaagacaaaatcagaacaagagagtatatatatatgtgtgtgtgtgtgtgtgtgtgtgtgtgtgtgtgtgtgtgtgtgtgactgggtcaccctgcggcacagcagaaattggcagaacattgtaaatcaactatactttaataggaaaaatacttttaagggctaaatttccaatattctaaccatgtacacagagtaaatgtcataaggatgccagtctgtgtagagattgatgtgttactagcagattcatgaaataaaggctgaggatgtagtccccaagtcacttctgagtggaagaatttctcctttgtcctggactcaaatattttaggataaaggaaaaaagaagatatttatagaagggacttgttttcaagtacttgacaaaatttcaccattaaagagaaatttgtgggagttcccatcgtggctcagtggaaacaaatccaactaggaaccatgaggttgtgggtttgatccctggcctcactcagtgggttaaggatccggtgttgccgtgagctgtggtgtaggttgcagacacggttctgatcctgcgttgctgtggctgtggctgtggtgtaggccagcagcaaacagctctgattagacccctagcctggaaacctccatatgccacaggtgcagccctaaaaagacaaaaaaagagaaaagacaaaaaaaaaaaaaaaaaaaaaaaaaaaaaaaaaaaaaaaaaaaagaacccccagaggtatttatttgtttttgccttttttcactgactgttctttgtttgtttgtttgagactgatctagaagactagagattacaagaaatatggatttggctcactctaagaaactgctttcattccaaggtttgggtctatccaaaagtggaatagaatcatatgaatactagtttatgagtatttagtgagaggaatttcaagctcaaataatgattcagcaagattaaattaaggagggaattttccttgtggctgagtgggttaaggacccaatgttgtctctgtgaggatgtaggttccatcctgggctttgctcattaggttaaggatctggcattgctgcagctcagacccagtgctgccctggttgtggcttaggccaaagctgcagctccaattcaatctctggcctgggaacctccatgtgctacaaggtgcggccttaaaaggaaaaaaaaaaaattaaatcaaggactcaagagtctttcattatttgtgttgtggaagctatatttgttttaaagtcttagttgtgtttagaaagcaagatgttcttcaactcaaatttgggagggaacttgtttcatacatttttaatggataagtggcaaaattttcatgctgaggtgatctatagtgttgtaatgcagaatatagtcagatcttgaacattttaggaagttggtgagggccaattgtgtatctgtgccatgctgataagaatgtcaagggatcacaagaattcgtgagctgtggtataggttgcagactctgctcaggtcccatgttgctgtgattgtggtgtaggctgactgctgcagcttcaatttgacccctagcccgggaatttccataggccacacgtgcagcactaaggaaggaaaaaaagaaaaaaaaaaaaaaagagtgggtgtgcctatagtgaagaacagatgtaaaagggaagtgaaagggattcccccattctgagggattgtgagaagtgtgccagaatattaacttcatttgacttgttacagggaaagtaaacttgactttcacggacctcctagttacctggtgcttactatatgtcttctcagagtacctgattcattcccagcctggttgacccatccccctatctctatggctatgtttatccagagcacatctatctaacactccagctgatcttcctgacacagctgtggcaaccctggatcctttaaccaactgtgccaggctggagatcaaacctaagcctctgcagcaacccaagctgctgcagtcagatttttaaccccctgtgccactgtgggtatctccgatattttgtatcttctgtgactgagtggtttgctgtttgcagggaaccagagtcagacactatccccgtgcaattcatcatcctcggacccatcaagctctattatttcagaagaaaatggtgttgcctgcataggtgagaatcagtgaccaacctatgaaaatgatctcaatcctctgaaatgcattttattcatgttttatttcctctttgcagggagtggtcaacttcgcctggtcgatggaggtggtcgttgtgctgggagagtagaggtctatcatgagggctcctggggcaccatctgtgatgacagctgggacctgaatgatgcccatgtggtgtgcaaacagctgagctgtggatgggccattaatgccactggttctgctcattttggggaaggaacagggcccatttggctggatgagataaactgtaatggaaaagaatctcatatttggcaatgccactcacatggttgggggcggcacaattgcaggcataaggaggatgcaggagtcatctgctcgg

SEQ ID NO: 110 - DNA, 3603 bp, Sus scrofa
tatagatgacaaggctttgtgtctgataggggccagcgaactcagtaaagagggaagatgagaaagataatggcaagaatttatccctgaagtgtagttttgacaaaccagtcacaaagaggtctaagaaattttggtcacaaagttgttttgaatcccaggcattttatttgcaatgattgcatatgttctggaaaggacatctgaacctaagaaatagttcatttgcattgtgttatattttactaaggtctgagaaataatcttgagatgagaatgaactctacttcttcagagtctggaaggaataaattatgaaaatgtattaatgcttctttaaaccatattgtatatttatctattactaaacaaaaagaagtagctctatttatttatttatttatttatttatttatgtcttttgtctctttagggccacacctgtggcatatggaggttcccaggctagaggtccaattggagatgttgtggagaattccacaagaattcgtgttatttgacagcagtcatctttaaaaggcatttgagaaagtccaatttcaaatgcatttcctttctttaaaagataaattgaagaaaataagtctttatttcccaagtaaattgaattgcctctcagtctgttaaaagaaactcttatatagatgacaaggctttgtgtctgataggggccagcgaactcagtaaagagggaagatgagaaagataatggcaagaatttatccctgaagtgtagttttgacaaaccagtcacaaagaggtctaagaaattttggtcacaaagttgttttgaatcccaggcattttatttgcaatgattgcatatgttctggaaaggacatctgaacctaagaaatagttcatttgcattgtgttatattttactaaggtctgagaaataatcttgagatgagaatgaactctacttcttcagagtctggaaggaataaattatgaaaatgtattaatgcttctttaaaccatattgtatatttatctattactaaacaaaaagaagtagctctatttatttatttatttatttatttatttatgtcttttgtctctttagggccacacctgtggcatatggaggttcccaggctagaggtccaattggagatgttgtggagaattccacaagaattcgtgttatttgacagcagtcatctttaaaaggcatttgagaaagtccaatttcaaatgcatttcctttctttaaaagataaattgaagaaaataagtctttatttcccaagtaaattgaattgcctctcagtctgttaaaagaaactcttaccttgatgattgcgctcttaacctggcaaagattgtctttaaaatctgagctccatgtcttctgctttatttctggtgtgcctttgactccagattacagtaaatggaggactgagtatagggctaaaaagtagagagaatggatgcatattatctgtggtctccaatgtgatgaatgaagtaggcaaatactcaaaggaaagagaaagcatgctccaagaattatgggttccagaaggcaaagtcccagaattgtctccagggaaggacagggaggtctagaatcggctaagcccactgtaggcagaaaaaccaagaggcatgaatggcttccctttctcacttttcactctctggcttactcctatcatgaaggaaaatattggaatcatattctccctcaccgaaatgctatttttcagcccacaggaaacccaggctggttggaggggacattccctgctctcactttggagaaggaagtggacagatctgggctgaagaattccagtgtgaggggcacgagtcccacctttcactctgcccagtagcaccccgccctgacgggacatgtagccacagcagggacgtcggcgtagtctgctcaagtgagacccagggaatgtgttcactttgttcccatgccatgaagagggtagggttaggtagtcacagacatctttttaaagccctgtctccttccaggatacacacaaatccgcttggtgaatggcaagaccccatgtgaaggaagagtggagctcaacattcttgggtcctgggggtccctctgcaactctcactgggacatggaagatgcccatgttttatgccagcagcttaaatgtggagttgccctttctatcccgggaggagcaccttttgggaaaggaagtgagcaggtctggaggcacatgtttcactgcactgggactgagaagcacatgggagattgttccgtcactgctctgggcgcatcactctgttcttcagggcaagtggcctctgtaatctgctcaggtaagagaataagggcagccagtgatgagccactcatgacggtgccttaagagtgggtgtacctaggagttcccattgtggctcagtggtaacaaactcgactggtatccatgagggtatgggtttgatccctggccttgctcaatgggttaaggatccagcattgctgtgagctgtggtataggttgcagactctgctcaggtcccatgttgctgtgattgtggtgtaggctgactgctgcagcttcaatttgacccctagcccgggaatttccataggccacacgtgcagcactaaggaaggaaaaaaagaaaaaaaaaaaaaaagagtgggtgtgcctatagtgaagaacagatgtaaaagggaagtgaaagggattcccccattctgagggattgtgagaagtgtgccagaatattaacttcatttgacttgttacagggaaagtaaacttgactttcacggacctcctagttacctggtgcttactatatgtcttctcagagtacctgattcattcccagcctggttgacccatccccctatctctatggctatgtttatccagagcacatctatctaacactccagctgatcttcctgacacagctgtggcaaccctggatcctttaaccaactgtgccaggctggagatcaaacctaagcctctgcagcaacccaagctgctgcagtcagatttttaaccccctgtgccactgtgggtatctccgatattttgtatcttctgtgactgagtggtttgctgtttgcagggaaccagagtcagacactatccccgtgcaattcatcatcctcggacccatcaagctctattatttcagaagaaaatggtgttgcctgcataggtgagaatcagtgaccaacctatgaaaatgatctcaatcctctgaaatgcattttattcatgttttatttcctctttgcagggagtggtcaacttcgcctggtcgatggaggtggtcgttgtgctgggagagtagaggtctatcatgagggctcctggggcaccatctgtgatgacagctgggacctgaatgatgcccatgtggtgtgcaaacagctgagctgtggatgggccattaatgccactggttctgctcattttggggaaggaacagggcccatttggctggatgagataaactgtaatggaaaagaatctcatatttggcaatgccactcacatggttgggggcggcacaattgcaggcataaggaggatgcaggagtcatctgctcgg

SEQ ID NO: 111 - DNA, 4962 bp, Sus scrofa
tatagatgacaaggctttgtgtctgataggggccagcgaactcagtaaagagggaagatgagaaagataatggcaagaatttatccctgaagtgtagttttgacaaaccagtcacaaagaggtctaagaaattttggtcacaaagttgttttgaatcccaggcattttatttgcaatgattgcatatgttctggaaaggacatctgaacctaagaaatagttcatttgcattgtgttatattttactaaggtctgagaaataatcttgagatgagaatgaactctacttcttcagagtctggaaggaataaattatgaaaatgtattaatgcttctttaaaccatattgtatatttatctattactaaacaaaaagaagtagctctatttatttatttatttatttatttatttatgtcttttgtctctttagggccacacctgtggcatatggaggttcccaggctagaggtccaattggagatgtagcagccagcctatgccagagccaccgcaacacgggatctgagccacgtctgtgacttacaccacagctcacagcaacgcctgatcctcaacccactgagcgaggccagggatcgaacccatgtcctcatggatgctagttgggttcgttaactgctgagccatgatgggaactccaaattaattatttcttatatttgttcttcatatattcatttctatagaaagaaataaatacagattcagttaatgatggcaggtaaaagcttaacttattaatcaaaggagttaatccaggcacaaaaattcaattcatggctctctgttaaaatttaggtataggtttagcaggaagaaaaggttagtagatgcagactattacatttagaatggatggacaatgaagtcctactatacagcacagggaactatatccaatctcttgggatagaatatgatggaagacaaaatcagaacaagagagtatatatatatgtgtgtgtgtgtgtgtgtgtgtgtgtgtgtgtgtgtgtgtgtgtgactgggtcaccctgcggcacagcagaaattggcagaacattgtaaatcaactatactttaataggaaaaatacttttaagggctaaatttccaatattctaaccatgtacacagagtaaatgtcataaggatgccagtctgtgtagagattgatgtgttactagcagattcatgaaataaaggctgaggatgtagtccccaagtcacttctgagtggaagaatttctcctttgtcctggactcaaatattttaggataaaggaaaaaagaagatatttatagaagggacttgttttcaagtacttgacaaaatttcaccattaaagagaaatttgtgggagttcccatcgtggctcagtggaaacaaatccaactaggaaccatgaggttgtgggtttgatccctggcctcactcagtgggttaaggatccggtgttgccgtgagctgtggtgtaggttgcagacacggttctgatcctgcgttgctgtggctgtggctgtggtgtaggccagcagcaaacagctctgattagacccctagcctggaaacctccatatgccacaggtgcagccctaaaaagacaaaaaaagagaaaagacaaaaaaaaaaaaaaaaaaaaaaaaaaaaaaaaaaaaaaaaaaaagaacccccagaggtatttatttgtttttgccttttttcactgactgttctttgtttgtttgtttgagactgatctagaagactagagattacaagaaatatggatttggctcactctaagaaactgctttcattccaaggtttgggtctatccaaaagtggaatagaatcatatgaatactagtttatgagtatttagtgagaggaatttcaagctcaaataatgattcagcaagattaaattaaggagggaattttccttgtggctgagtgggttaaggacccaatgttgtctctgtgaggatgtaggttccatcctgggctttgctcattaggttaaggatctggcattgctgcagctcagacccagtgctgccctggttgtggcttaggccaaagctgcagctccaattcaatctctggcctgggaacctccatgtgctacaaggtgcggccttaaaaggaaaaaaaaaaaattaaatcaaggactcaagagtctttcattatttgtgttgtggaagctatatttgttttaaagtcttagttgtgtttagaaagcaagatgttcttcaactcaaatttgggagggaacttgtttcatacatttttaatggataagtggcaaaattttcatgctgaggtgatctatagtgttgtaatgcagaatatagtcagatcttgaacattttaggaagttggtgagggccaattgtgtatctgtgccatgctgataagaatgtcaagggatcacaagaattcgtgttatttgacagcagtcatctttaaaaggcatttgagaaagtccaatttcaaatgcatttcctttctttaaaagataaattgaagaaaataagtctttatttcccaagtaaattgaattgcctctcagtctgttaaaagaaactcttaccttgatgattgcgctcttaacctggcaaagattgtctttaaaatctgagctccatgtcttctgctttatttctggtgtgcctttgactccagattacagtaaatggaggactgagtatagggctaaaaagtagagagaatggatgcatattatctgtggtctccaatgtgatgaatgaagtaggcaaatactcaaaggaaagagaaagcatgctccaagaattatgggttccagaaggcaaagtcccagaattgtctccagggaaggacagggaggtctagaatcggctaagcccactgtaggcagaaaaaccaagaggcatgaatggcttccctttctcacttttcactctctggcttactcctatcatgaaggaaaatattggaatcatattctccctcaccgaaatgctatttttcagcccacaggaaacccaggctggttggaggggacattccctgctctggtcgtgttgaagtacaacatggagacacgtggggcaccgtctgtgattctgacttctctctggaggcggccagcgtgctgtgcagggaactacagtgcgtcactttggagaaggaagtggacagatctgggctgaagaattccagtgtgaggggcacgagtcccacctttcactctgcccagtagcaccccgccctgacgggacatgtagccacagcagggacgtcggcgtagtctgctcaagtgagacccagggaatgtgttcactttgttcccatgccatgaagagggtagggttaggtagtcacagacatctttttaaagccctgtctccttccaggatacacacaaatccgcttggtgaatggcaagaccccatgtgaaggaagagtggagctcaacattcttgggtcctgggggtccctctgcaactctcactgggacatggaagatgcccatgttttatgccagcagcttaaatgtggagttgccctttctatcccgggaggagcaccttttgggaaaggaagtgagcaggtctggaggcacatgtttcactgcactgggactgagaagcacatgggagattgttccgtcactgctctgggcgcatcactctgttcttcagggcaagtggcctctgtaatctgctcaggtaagagaataagggcagccagtgatgagccactcatgacggtgccttaagagtgggtgtacctaggagttcccattgtggctcagtggtaacaaactcgactggtatccatgagggtatgggtttgatccctggccttgctcaatgggttaaggatccagcattgctgtgagctgtggtataggttgcagactctgctcaggtcccatgttgctgtgattgtggtgtaggctgactgctgcagcttcaatttgacccctagcccgggaatttccataggccacacgtgcagcactaaggaaggaaaaaaagaaaaaaaaaaaaaaagagtgggtgtgcctatagtgaagaacagatgtaaaagggaagtgaaagggattcccccattctgagggattgtgagaagtgtgccagaatattaacttcatttgacttgttacagggaaagtaaacttgactttcacggacctcctagttacctggtgcttactatatgtcttctcagagtacctgattcattcccagcctggttgacccatccccctatctctatggctatgtttatccagagcacatctatctaacactccagctgatcttcctgacacagctgtggcaaccctggatcctttaaccaactgtgccaggctggagatcaaacctaagcctctgcagcaacccaagctgctgcagtcagatttttaaccccctgtgccactgtgggtatctccgatattttgtatcttctgtgactgagtggtttgctgtttgcagggaaccagagtcagacactatccccgtgcaattcatcatcctcggacccatcaagctctattatttcagaagaaaatggtgttgcctgcataggtgagaatcagtgaccaacctatgaaaatgatctcaatcctctgaaatgcattttattcatgttttatttcctctttgcagggagtggtcaacttcgcctggtcgatggaggtggtcgttgtgctgggagagtagaggtctatcatgagggctcctggggcaccatctgtgatgacagctgggacctgaatgatgcccatgtggtgtgcaaacagctgagctgtggatgggccattaatgccactggttctgctcattttggggaaggaacagggcccatttggctggatgagataaactgtaatggaaaagaatctcatatttggcaatgccactcacatggttgggggcggcacaattgcaggcataaggaggatgcaggagtcatctgctcgg

SEQ ID NO: 112 - DNA, 3603 bp, Sus scrofa
tatagatgacaaggctttgtgtctgataggggccagcgaactcagtaaagagggaagatgagaaagataatggcaagaatttatccctgaagtgtagttttgacaaaccagtcacaaagaggtctaagaaattttggtcacaaagttgttttgaatcccaggcattttatttgcaatgattgcatatgttctggaaaggacatctgaacctaagaaatagttcatttgcattgtgttatattttactaaggtctgagaaataatcttgagatgagaatgaactctacttcttcagagtctggaaggaataaattatgaaaatgtattaatgcttctttaaaccatattgtatatttatctattactaaacaaaaagaagtagctctatttatttatttatttatttatttatttatgtcttttgtctctttagggccacacctgtggcatatggaggttcccaggctagaggtccaattggagatgtagcagccagcctatgccagagccaccgcaacacgggatctgagccacgtctgtgacttacaccacagctcacagcaacgcctgatcctcaacccactgagcgaggccagggatcgaacccatgtcctcatggatgctagttgggttcgttaactgctgagccatgatgggaactccaaattaattatttcttatatttgttcttcatatattcatttctatagaaagaaataaatacagattcagttaatgatggcaggtaaaagcttaacttattaatcaaaggagttaatccaggcacaaaaattcaattcatggctctctgttaaaatttaggtataggtttagcaggaagaaaaggttagtagatgcagactattacatttagaatggatggacaatgaagtcctactatacagcacagggaactatatccaatctcttgggatagaatatgatggaagacaaaatcagaacaagagagtatatatatatgtgtgtgtgtgtgtgtgtgtgtgtgtgtgtgtgtgtgtgtgtgtgactgggtcaccctgcggcacagcagaaattggcagaacattgtaaatcaactatactttaataggaaaaatacttttaagggctaaatttccaatattctaaccatgtacacagagtaaatgtcataaggatgccagtctgtgtagagattgatgtgttactagcagattcatgaaataaaggctgaggatgtagtccccaagtcacttctgagtggaagaatttctcctttgtcctggactcaaatattttaggataaaggaaaaaagaagatatttatagaagggacttgttttcaagtacttgacaaaatttcaccattaaagagaaatttgtgggagttcccatcgtggctcagtggaaacaaatccaactaggaaccatgaggttgtgggtttgatccctggcctcactcagtgggttaaggatccggtgttgccgtgagctgtggtgtaggttgcagacacggttctgatcctgcgttgctgtggctgtggctgtggtgtaggccagcagcaaacagctctgattagacccctagcctggaaacctccatatgccacaggtgcagccctaaaaagacaaaaaaagagaaaagacaaaaaaaaaaaaaaaaaaaaaaaaaaaaaaaaaaaaaaaaaaaagaacccccagaggtatttatttgtttttgccttttttcactgactgttctttgtttgtttgtttgagactgatctagaagactagagattacaagaaatatggatttggctcactctaagaaactgctttcattccaaggtttgggtctatccaaaagtggaatagaatcatatgaatactagtttatgagtatttagtgagaggaatttcaagctcaaataatgattcagcaagattaaattaaggagggaattttccttgtggctgagtgggttaaggacccaatgttgtctctgtgaggatgtaggttccatcctgggctttgctcattaggttaaggatctggcattgctgcagctcagacccagtgctgccctggttgtggcttaggccaaagctgcagctccaattcaatctctggcctgggaacctccatgtgctacaaggtgcggccttaaaaggaaaaaaaaaaaattaaatcaaggactcaagagtctttcattatttgtgttgtggaagctatatttgttttaaagtcttagttgtgtttagaaagcaagatgttcttcaactcaaatttgggagggaacttgtttcatacatttttaatggataagtggcaaaattttcatgctgaggtgatctatagtgttgtaatgcagaatatagtcagatcttgaacattttaggaagttggtgagggccaattgtgtatctgtgccatgctgataagaatgtcaagggatcacaagaattcgtgttatttgacagcagtcatctttaaaaggcatttgagaaagtccaatttcaaatgcatttcctttctttaaaagataaattgaagaaaataagtctttatttcccaagtaaattgaattgcctctcagtctgttaaaagaaactcttaccttgatgattgcgctcttaacctggcaaagattgtctttaaaatctgagctccatgtcttctgctttatttctggtgtgcctttgactccagattacagtaaatggaggactgagtatagggctaaaaagtagagagaatggatgcatattatctgtggtctccaatgtgatgaatgaagtaggcaaatactcaaaggaaagagaaagcatgctccaagaattatgggttccagaaggcaaagtcccagaattgtctccagggaaggacagggaggtctagaatcggctaagcccactgtaggcagaaaaaccaagaggcatgaatggcttccctttctcacttttcactctctggcttactcctatcatgaaggaaaatattggaatcatattctccctcaccgaaatgctatttttcagcccacaggaaacccaggctggttggaggggacattccctgctctggtcgtgttgaagtacaacatggagacacgtggggcaccgtctgtgattctgacttctctctggaggcggccagcgtgctgtgcagggaactacagtgcgattcatcatcctcggacccatcaagctctattatttcagaagaaaatggtgttgcctgcataggtgagaatcagtgaccaacctatgaaaatgatctcaatcctctgaaatgcattttattcatgttttatttcctctttgcagggagtggtcaacttcgcctggtcgatggaggtggtcgttgtgctgggagagtagaggtctatcatgagggctcctggggcaccatctgtgatgacagctgggacctgaatgatgcccatgtggtgtgcaaacagctgagctgtggatgggccattaatgccactggttctgctcattttggggaaggaacagggcccatttggctggatgagataaactgtaatggaaaagaatctcatatttggcaatgccactcacatggttgggggcggcacaattgcaggcataaggaggatgcaggagtcatctgctcgg

SEQ ID NO: 113 - DNA, 3619 bp, Sus scrofa
tatagatgacaaggctttgtgtctgataggggccagcgaactcagtaaagagggaagatgagaaagataatggcaagaatttatccctgaagtgtagttttgacaaaccagtcacaaagaggtctaagaaattttggtcacaaagttgttttgaatcccaggcattttatttgcaatgattgcatatgttctggaaaggacatctgaacctaagaaatagttcatttgcattgtgttatattttactaaggtctgagaaataatcttgagatgagaatgaactctacttcttcagagtctggaaggaataaattatgaaaatgtattaatgcttctttaaaccatattgtatatttatctattactaaacaaaaagaagtagctctatttatttatttatttatttatttatttatgtcttttgtctctttagggccacacctgtggcatatggaggttcccaggctagaggtccaattggagatgtagcagccagcctatgccagagccaccgcaacacgggatctgagccacgtctgtgacttacaccacagctcacagcaacgcctgatcctcaacccactgagcgaggccagggatcgaacccatgtcctcatggatgctagttgggttcgttaactgctgagccatgatgggaactccaaattaattatttcttatatttgttcttcatatattcatttctatagaaagaaataaatacagattcagttaatgatggcaggtaaaagcttaacttattaatcaaaggagttaatccaggcacaaaaattcaattcatggctctctgttaaaatttaggtataggtttagcaggaagaaaaggttagtagatgcagactattacatttagaatggatggacaatgaagtcctactatacagcacagggaactatatccaatctcttgggatagaatatgatggaagacaaaatcagaacaagagagtatatatatatgtgtgtgtgtgtgtgtgtgtgtgtgtgtgtgtgtgtgtgtgtgtgactgggtcaccctgcggcacagcagaaattggcagaacattgtaaatcaactatactttaataggaaaaatacttttaagggctaaatttccaatattctaaccatgtacacagagtaaatgtcataaggatgccagtctgtgtagagattgatgtgttactagcagattcatgaaataaaggctgaggatgtagtccccaagtcacttctgagtggaagaatttctcctttgtcctggactcaaatattttaggataaaggaaaaaagaagatatttatagaagggacttgttttcaagtacttgacaaaatttcaccattaaagagaaatttgtgggagttcccatcgtggctcagtggaaacaaatccaactaggaaccatgaggttgtgggtttgatccctggcctcactcagtgggttaaggatccggtgttgccgtgagctgtggtgtaggttgcagacacggttctgatcctgcgttgctgtggctgtggctgtggtgtaggccagcagcaaacagctctgattagacccctagcctggaaacctccatatgccacaggtgcagccctaaaaagacaaaaaaagagaaaagacaaaaaaaaaaaaaaaaaaaaaaaaaaaaaaaaaaaaaaaaaaaagaacccccagaggtatttatttgtttttgccttttttcactgactgttctttgtttgtttgtttgagactgatctagaagactagagattacaagaaatatggatttggctcactctaagaaactgctttcattccaaggtttgggtctatccaaaagtggaatagaatcatatgaatactagtttatgagtatttagtgagaggaatttcaagctcaaataatgattcagcaagattaaattaaggagggaattttccttgtggctgagtgggttaaggacccaatgttgtctctgtgaggatgtaggttccatcctgggctttgctcattaggttaaggatctggcattgctgcagctcagacccagtgctgccctggttgtggcttaggccaaagctgcagctccaattcaatctctggcctgggaacctccatgtgctacaaggtgcggccttaaaaggaaaaaaaaaaaattaaatcaaggactcaagagtctttcattatttgtgttgtggaagctatatttgttttaaagtcttagttgtgtttagaaagcaagatgttcttcaactcaaatttgggagggaacttgtttcatacatttttaatggataagtggcaaaattttcatgctgaggtgatctatagtgttgtaatgcagaatatagtcagatcttgaacattttaggaagttggtgagggccaattgtgtatctgtgccatgctgataagaatgtcaagggatcacaagaattcgtgttatttgacagcagtcatctttaaaaggcatttgagaaagtccaatttcaaatgcatttcctttctttaaaagataaattgaagaaaataagtctttatttcccaagtaaattgaattgcctctcagtctgttaaaagaaactcttaccttgatgattgcgctcttaacctggcaaagattgtctttaaaatctgagctccatgtcttctgctttatttctggtgtgcctttgactccagattacagtaaatggaggactgagtatagggctaaaaagtagagagaatggatgcatattatctgtggtctccaatgtgatgaatgaagtaggcaaatactcaaaggaaagagaaagcatgctccaagaattatgggttccagaaggcaaagtcccagaattgtctccagggaaggacagggaggtctagaatcggctaagcccactgtaggcagaaaaaccaagaggcatgaatggcttccctttctcacttttcactctctggcttactcctatcatgaaggaaaatattggaatcatattctccctcaccgaaatgctatttttcagcccacaggaaacccaggctggttggaggggacattccctgctctggtcgtgttgaagtacaacatggagacacgtggggcaccgtctgtgattctgacttctctctggaggcagccagcgtgctttgcagggaaccagagtcagacactatccccgtgcaattcatcatcctcggacccatcaagctctattatttcagaagaaaatggtgttgcctgcataggtgagaatcagtgaccaacctatgaaaatgatctcaatcctctgaaatgcattttattcatgttttatttcctctttgcagggagtggtcaacttcgcctggtcgatggaggtggtcgttgtgctgggagagtagaggtctatcatgagggctcctggggcaccatctgtgatgacagctgggacctgaatgatgcccatgtggtgtgcaaacagctgagctgtggatgggccattaatgccactggttctgctcattttggggaaggaacagggcccatttggctggatgagataaactgtaatggaaaagaatctcatatttggcaatgccactcacatggttgggggcggcacaattgcaggcataaggaggatgcaggagtcatctgctcgg

SEQ ID NO: 114 - DNA, 3270 bp, Sus scrofa
tatagatgacaaggctttgtgtctgataggggccagcgaactcagtaaagagggaagatgagaaagataatggcaagaatttatccctgaagtgtagttttgacaaaccagtcacaaagaggtctaagaaattttggtcacaaagttgttttgaatcccaggcattttatttgcaatgattgcatatgttctggaaaggacatctgaacctaagaaatagttcatttgcattgtgttatattttactaaggtctgagaaataatcttgagatgagaatgaactctacttcttcagagtctggaaggaataaattatgaaaatgtattaatgcttctttaaaccatattgtatatttatctattactaaacaaaaagaagtagctctatttatttatttatttatttatttatttatgtcttttgtctctttagggccacacctgtggcatatggaggttcccaggctagaggtccaattggagatgtagcagccagcctatgccagagccaccgcaacacgggatctgagccacgtctgtgacttacaccacagctcacagcaacgcctgatcctcaacccactgagcgaggccagggatcgaacccatgtcctcatggatgctagttgggttcgttaactgctgagccatgatgggaactccaaattaattatttcttatatttgttcttcatatattcatttctatagaaagaaataaatacagattcagttaatgatggcaggtaaaagcttaacttattaatcaaaggagttaatccaggcacaaaaattcaattcatggctctctgttaaaatttaggtataggtttagcaggaagaaaaggttagtagatgcagactattacatttagaatggatggacaatgaagtcctactatacagcacagggaactatatccaatctcttgggatagaatatgatggaagacaaaatcagaacaagagagtatatatatatgtgtgtgtgtgtgtgtgtgtgtgtgtgtgtgtgtgtgtgtgtgtgactgggtcaccctgcggcacagcagaaattggcagaacattgtaaatcaactatactttaataggaaaaatacttttaagggctaaatttccaatattctaaccatgtacacagagtaaatgtcataaggatgccagtctgtgtagagattgatgtgttactagcagattcatgaaataaaggctgaggatgtagtccccaagtcacttctgagtggaagaatttctcctttgtcctggactcaaatattttaggataaaggaaaaaagaagatatttatagaagggacttgttttcaagtacttgacaaaatttcaccattaaagagaaatttgtgggagttcccatcgtggctcagtggaaacaaatccaactaggaaccatgaggttgtgggtttgatccctggcctcactcagtgggttaaggatccggtgttgccgtgagctgtggtgtaggttgcagacacggttctgatcctgcgttgctgtggctgtggctgtggtgtaggccagcagcaaacagctctgattagacccctagcctggaaacctccatatgccacaggtgcagccctaaaaagacaaaaaaagagaaaagacaaaaaaaaaaaaaaaaaaaaaaaaaaaaaaaaaaaaaaaaaaaagaacccccagaggtatttatttgtttttgccttttttcactgactgttctttgtttgtttgtttgagactgatctagaagactagagattacaagaaatatggatttggctcactctaagaaactgctttcattccaaggtttgggtctatccaaaagtggaatagaatcatatgaatactagtttatgagtatttagtgagaggaatttcaagctcaaataatgattcagcaagattaaattaaggagggaattttccttgtggctgagtgggttaaggacccaatgttgtctctgtgaggatgtaggttccatcctgggctttgctcattaggttaaggatctggcattgctgcagctcagacccagtgctgccctggttgtggcttaggccaaagctgcagctccaattcaatctctggcctgggaacctccatgtgctacaaggtgcggccttaaaaggaaaaaaaaaaaattaaatcaaggactcaagagtctttcattatttgtgttgtggaagctatatttgttttaaagtcttagttgtgtttagaaagcaagatgttcttcaactcaaatttgggagggaacttgtttcatacatttttaatggataagtggcaaaattttcatgctgaggtgatctatagtgttgtaatgcagaatatagtcagatcttgaacattttaggaagttggtgagggccaattgtgtatctgtgccatgctgataagaatgtcaagggatcacaagaattcgtgttatttgacttgttacagggaaagtaaacttgactttcacggacctcctagttacctggtgcttactatatgtcttctcagagtacctgattcattcccagcctggttgacccatccccctatctctatggctatgtttatccagagcacatctatctaacactccagctgatcttcctgacacagctgtggcaaccctggatcctttaaccaactgtgccaggctggagatcaaacctaagcctctgcagcaacccaagctgctgcagtcagatttttaaccccctgtgccactgtgggtatctccgatattttgtatcttctgtgactgagtggtttgctgtttgcagggaaccagagtcagacactatccccgtgcaattcatcatcctcggacccatcaagctctattatttcagaagaaaatggtgttgcctgcataggtgagaatcagtgaccaacctatgaaaatgatctcaatcctctgaaatgcattttattcatgttttatttcctctttgcagggagtggtcaacttcgcctggtcgatggaggtggtcgttgtgctgggagagtagaggtctatcatgagggctcctggggcaccatctgtgatgacagctgggacctgaatgatgcccatgtggtgtgcaaacagctgagctgtggatgggccattaatgccactggttctgctcattttggggaaggaacagggcccatttggctggatgagataaactgtaatggaaaagaatctcatatttggcaatgccactcacatggttgggggcggcacaattgcaggcataaggaggatgcaggagtcatctgctcgg

SEQ ID NO: 115 - DNA, 7 bp, Sus scrofa
tactact

SEQ ID NO: 116 - DNA, 12 bp, Sus scrofa
tgtggagaattc

SEQ ID NO: 117 - DNA, 11 bp, Sus scrofa
agccagcgtgc

SEQ ID NO: 118 - DNA, 8532 bp, Sus scrofa
tatagatgacaaggctttgtgtctgataggggccagcgaactcagtaaagagggaagatgagaaagataatggcaagaatttatccctgaagtgtagttttgacaaaccagtcacaaagaggtctaagaaattttggtcacaaagttgttttgaatcccaggcattttatttgcaatgattgcatatgttctggaaaggacatctgaacctaagaaatagttcatttgcattgtgttatattttactaaggtctgagaaataatcttgagatgagaatgaactctacttcttcagagtctggaaggaataaattatgaaaatgtattaatgcttctttaaaccatattgtatatttatctattactaaacaaaaagaagtagctctatttatttatttatttatttatttatttatgtcttttgtctctttagggccacacctgtggcatatggaggttcccaggctagaggtccaattggagatgtagcagccagcctatgccagagccaccgcaacacgggatctgagccacgtctgtgacttacaccacagctcacagcaacgcctgatcctcaacccactgagcgaggccagggatcgaacccatgtcctcatggatgctagttgggttcgttaactgctgagccatgatgggaactccaaattaattatttcttatatttgttcttcatatattcatttctatagaaagaaataaatacagattcagttaatgatggcaggtaaaagcttaacttattaatcaaaggagttaatccaggcacaaaaattcaattcatggctctctgttaaaatttaggtataggtttagcaggaagaaaaggttagtagatgcagactattacatttagaatggatggacaatgaagtcctactatacagcacagggaactatatccaatctcttgggatagaatatgatggaagacaaaatcagaacaagagagtatatatatatgtgtgtgtgtgtgtgtgtgtgtgtgtgtgtgtgtgtgtgtgtgtgactgggtcaccctgcggcacagcagaaattggcagaacattgtaaatcaactatactttaataggaaaaatacttttaagggctaaatttccaatattctaaccatgtacacagagtaaatgtcataaggatgccagtctgtgtagagattgatgtgttactagcagattcatgaaataaaggctgaggatgtagtccccaagtcacttctgagtggaagaatttctcctttgtcctggactcaaatattttaggataaaggaaaaaagaagatatttatagaagggacttgttttcaagtacttgacaaaatttcaccattaaagagaaatttgtgggagttcccatcgtggctcagtggaaacaaatccaactaggaaccatgaggttgtgggtttgatccctggcctcactcagtgggttaaggatccggtgttgccgtgagctgtggtgtaggttgcagacacggttctgatcctgcgttgctgtggctgtggctgtggtgtaggccagcagcaaacagctctgattagacccctagcctggaaacctccatatgccacaggtgcagccctaaaaagacaaaaaaagagaaaagacaaaaaaaaaaaaaaaaaaaaaaaaaaaaaaaaaaaaaaaaaaaagaacccccagaggtatttatttgtttttgccttttttcactgactgttctttgtttgtttgtttgagactgatctagaagactagagattacaagaaatatggatttggctcactctaagaaactgctttcattccaaggtttgggtctatccaaaagtggaatagaatcatatgaatactagtttatgagtatttagtgagaggaatttcaagctcaaataatgattcagcaagattaaattaaggagggaattttccttgtggctgagtgggttaaggacccaatgttgtctctgtgaggatgtaggttccatcctgggctttgctcattaggttaaggatctggcattgctgcagctcagacccagtgctgccctggttgtggcttaggccaaagctgcagctccaattcaatctctggcctgggaacctccatgtgctacaaggtgcggccttaaaaggaaaaaaaaaaaattaaatcaaggactcaagagtctttcattatttgtgttgtggaagctatatttgttttaaagtcttagttgtgtttagaaagcaagatgttcttcaactcaaatttgggagggaacttgtttcatacatttttaatggataagtggcaaaattttcatgctgaggtgatctatagtgttgtaatgcagaatatagtcagatcttgaacattttaggaagttggtgagggccaattgtgtatctgtgccatgctgataagaatgtcaagggatcacaagaattcgtgttatttgacagcagtcatctttaaaaggcatttgagaaagtccaatttcaaatgcatttcctttctttaaaagataaattgaagaaaataagtctttatttcccaagtaaattgaattgcctctcagtctgttaaaagaaactcttaccttgatgattgcgctcttaacctggcaaagattgtctttaaaatctgagctccatgtcttctgctttatttctggtgtgcctttgactccagattacagtaaatggaggactgagtatagggctaaaaagtagagagaatggatgcatattatctgtggtctccaatgtgatgaatgaagtaggcaaatactcaaaggaaagagaaagcatgctccaagaattatgggttccagaaggcaaagtcccagaattgtctccagggaaggacagggaggtctagaatcggctaagcccactgtaggcagaaaaaccaagaggcatgaatggcttccctttctcacttttcactctctggcttactcctatcatgaaggaaaatattggaatcatattctccctcaccgaaatgctatttttcagcccacaggaaacccaggctggttggagctgacatgccctgctctggtcgtgttgaagtaaaacatgcagacacgtggggctccgtctgtgattctgacttctctctgcatgcggccaacgtgctgtgcagggaactaaattgcggcgatgcgatttccctctcggtgggagatcactttggaaaaggaaatggactgacctgggctgaaaaattccagtgtgaggggagcgagacccaccttgcactctgcccaatagtacaacaccctgaagacacatgtatccacagcagggaagtcggcgtagtctgctcaagtaagagtttactgaaaataacactcttaaaatcttgttatgtttttattcataatgtgaatgagtagtagtggaaaataactaccagtttcctaagcttataacttcgtatagcatacattatacgaagttataagcctgcaggaattctaccgggtaggggaggcgcttttcccaaggcagtctggagcatgcgctttagcagccccgctgggcacttggcgctacacaagtggcctctggcctcgcacacattccacatccaccggtaggcgccaaccggctccgttctttggtggccccttcgcgccaccttctactcctcccctagtcaggaagttcccccccgccccgcagctcgcgtcgtgcaggacgtgacaaatggaagtagcacgtctcactagtctcgtgcagatggacagcaccgctgagcaatggaagcgggtaggcctttggggcagcggccaatagcagctttgctccttcgctttctgggctcagaggctgggaaggggtgggtccgggggcgggctcaggggcgggctcaggggcggggcgggcgcccgaaggtcctccggaggcccggcattctgcacgcttcaaaagcgcacgtctgccgcgctgttctcctcttcctcatctccgggcctttcgacctgcagccaccatggccatgattgaacaggatggcctgcatgcaggttctccagctgcctgggtggagagactgtttggctatgactgggcacagcagaccattggttgctctgatgcagcagtgttcagactgtcagcccagggcaggccagtcctgtttgtgaagacagacctcagtggggctctcaatgagctgcaggatgaggctgccagactctcctggctggcaacaactggggtcccctgtgcagctgtcctggatgtggtcacagaagctggaagggactggctcctgctgggtgaggtgcctgggcaggacctcctgtcctctcacctggctccagctgagaaagtgtcaatcatggctgatgccatgagaagactccacaccctggacccagccacctgcccctttgaccaccaggccaagcacaggattgagagggccagaaccaggatggaggctggcctggtggaccaggatgacctggatgaagaacaccagggcctggcccctgctgaactgtttgccaggctcaaggcatccatgccagatggtgaggacctggtggtgactcatggggatgcctgcctgcccaacatcatggtggaaaatggaaggttctctggcttcattgactgtggcaggctgggagtggctgacaggtaccaggacattgccctggcaaccagggacattgcagaagagctggggggagaatgggcagacaggttcctggtgctctatggcattgcagcccctgactcccagagaattgccttctacagactgctggatgagttcttctaaatcgattataatcagccataccacatttgtagaggttttacttgctttaaaaaacctcccacacctccccctgaacctgaaacataaaatgaatgcaatgttgttgttaaacttgtttattgcagcttataatggttacaaataaagcaatagcatcacaaatttcacaaataaagcatttttttcactgcattctagttgtggtttgtccaaactcatcaatgtggaaaataactaccagtttcctaagcttataacttcgtatagcatacattatacgaagttataagctagacaaaagtatcttaccccaatggtagccctgtacccaataaaagtaggtgttcagtttcatatcctatgaaataccctcttgatacttttactttgcatgaggatttagaagaaaaaagttttactataatccttaacttaggaaattcttttgaattggaaatgaaacacaaattgcttttcattgatatgccatatgattatatgaataaaacatgaaatcttcatattggattctagtatatacccaagtaaatattttttccctagaagagtgccaagtgtgttaaaaccttttggtttaataaagcagaaaaaaataaactctaaaaatcataattaaaaatgaaatgcttttatttatagcaattaactacaacatgtttagacttacatactattaaatataatatatttaagatcccctcatgataaatatgttcattattttgtaggctgttgatgcactaatatgtatgtagattactttgtgaattgcccttaataaaatttaaaactttaggctagtaaacctgtaacactcaacttagttctgaactatctcactattcttttgcaagaatttacttaggtaatgccaactaatttattccaaggccaaaaagatgacaatgtcttatatattataaaaactaataaaaaccattttaaaacctagtataaatttaaaggtacttgctcttctggttcatctcttcttttgtttacttctgctttcaaaaacttatttattgtgaccatattctttacttccatttattgttataatttataagatactatacttgcaagcaataaatgttatctttttagcttttaaatggtctcatttgaaaagaatatataattagtaagtcatagctactttaaataaaaacttattctttaagagattaaacacttctccaagtgatctgtttttctttaattaaaacgttattaactcccaaaatgatgttattgtttttttataatcttaaataccaataattaccaggtctattttgattttgatacaggataaaaactactattaattacttaagaatgtgttcttttttatatgtaccattttcatgatcaaagttggtgatatgactgaggttttgattattattaaacagatagttaatatgatatattcctcatttttccaaatgaaaggaaaaatgtcttatatggaggaaaagattggggcagggggattagtaaattattacttaaatatctgaataggaggatttttcaatgaaaggataaaggaagaatgattgtatcatctgaatctttccctccctttcctggagtttgtcctttcaacccagtatacctaccactcccttcatcacctactttcccattacagtccctatgtgttgggtggtaactattttgttttggtgttaatatccaagtttcccttaataacacctagtgaatggaggaaggatgagcatacctacccatcagacatatttagccaccatatttaatcaacaagcatgaagaaaggaagctagcctctccccttcctttcctcctgcctctctctctcttctctgtcctcgctccctttcttcccatcaatattttcagagcacctcttatgcgccaggcattgggatactcaaactggaggaaacaagaaaaaaaaaaaaaaaaggcgaagacctcagggaaatttatattgctgctatatttttttgagcctagtgtaaattaaaattccttaatgctgtgccttttaaaaacacaaataagcaaaatagtttatttcttcaacagttaaatccttagggtaggaaagtgattcaggatctattgctactattaactcttctttcattttcacacaggatacacacaaatccgcttggtgaatggcaagaccccatgtgaaggaagagtggagctcaacattcttgggtcctgggggtccctctgcaactctcactgggacatggaagatgcccatgttttatgccagcagcttaaatgtggagttgccctttctatcccgggaggagcaccttttgggaaaggaagtgagcaggtctggaggcacatgtttcactgcactgggactgagaagcacatgggagattgttccgtcactgctctgggcgcatcactctgttcttcagggcaagtggcctctgtaatctgctcaggtaagagaataagggcagccagtgatgagccactcatgacggtgccttaagagtgggtgtacctaggagttcccattgtggctcagtggtaacaaactcgactggtatccatgagggtatgggtttgatccctggccttgctcaatgggttaaggatccagcattgctgtgagctgtggtataggttgcagactctgctcaggtcccatgttgctgtgattgtggtgtaggctgactgctgcagcttcaatttgacccctagcccgggaatttccataggccacacgtgcagcactaaggaaggaaaaaaagaaaaaaaaaaaaaaagagtgggtgtgcctatagtgaagaacagatgtaaaagggaagtgaaagggattcccccattctgagggattgtgagaagtgtgccagaatattaacttcatttgacttgttacagggaaagtaaacttgactttcacggacctcctagttacctggtgcttactatatgtcttctcagagtacctgattcattcccagcctggttgacccatccccctatctctatggctatgtttatccagagcacatctatctaacactccagctgatcttcctgacacagctgtggcaaccctggatcctttaaccaactgtgccaggctggagatcaaacctaagcctctgcagcaacccaagctgctgcagtcagatttttaaccccctgtgccactgtgggtatctccgatattttgtatcttctgtgactgagtggtttgctgtttgcagggaaccagagtcagacactatccccgtgcaattcatcatcctcggacccatcaagctctattatttcagaagaaaatggtgttgcctgcataggtgagaatcagtgaccaacctatgaaaatgatctcaatcctctgaaatgcattttattcatgttttatttcctctttgcagggagtggtcaacttcgcctggtcgatggaggtggtcgttgtgctgggagagtagaggtctatcatgagggctcctggggcaccatctgtgatgacagctgggacctgaatgatgcccatgtggtgtgcaaacagctgagctgtggatgggccattaatgccactggttctgctcattttggggaaggaacagggcccatttggctggatgagataaactgtaatggaaaagaatctcatatttggcaatgccactcacatggttgggggcggcacaattgcaggcataaggaggatgcaggagtcatctgctcgg

SEQ ID NO: 119 - DNA, 4538 bp, Sus scrofa
tatagatgacaaggctttgtgtctgataggggccagcgaactcagtaaagagggaagatgagaaagataatggcaagaatttatccctgaagtgtagttttgacaaaccagtcacaaagaggtctaagaaattttggtcacaaagttgttttgaatcccaggcattttatttgcaatgattgcatatgttctggaaaggacatctgaacctaagaaatagttcatttgcattgtgttatattttactaaggtctgagaaataatcttgagatgagaatgaactctacttcttcagagtctggaaggaataaattatgaaaatgtattaatgcttctttaaaccatattgtatatttatctattactaaacaaaaagaagtagctctatttatttatttatttatttatttatttatgtcttttgtctctttagggccacacctgtggcatatggaggttcccaggctagaggtccaattggagatgtagcagccagcctatgccagagccaccgcaacacgggatctgagccacgtctgtgacttacaccacagctcacagcaacgcctgatcctcaacccactgagcgaggccagggatcgaacccatgtcctcatggatgctagttgggttcgttaactgctgagccatgatgggaactccaaattaattatttcttatatttgttcttcatatattcatttctatagaaagaaataaatacagattcagttaatgatggcaggtaaaagcttaacttattaatcaaaggagttaatccaggcacaaaaattcaattcatggctctctgttaaaatttaggtataggtttagcaggaagaaaaggttagtagatgcagactattacatttagaatggatggacaatgaagtcctactatacagcacagggaactatatccaatctcttgggatagaatatgatggaagacaaaatcagaacaagagagtatatatatatgtgtgtgtgtgtgtgtgtgtgtgtgtgtgtgtgtgtgtgtgtgtgactgggtcaccctgcggcacagcagaaattggcagaacattgtaaatcaactatactttaataggaaaaatacttttaagggctaaatttccaatattctaaccatgtacacagagtaaatgtcataaggatgccagtctgtgtagagattgatgtgttactagcagattcatgaaataaaggctgaggatgtagtccccaagtcacttctgagtggaagaatttctcctttgtcctggactcaaatattttaggataaaggaaaaaagaagatatttatagaagggacttgttttcaagtacttgacaaaatttcaccattaaagagaaatttgtgggagttcccatcgtggctcagtggaaacaaatccaactaggaaccatgaggttgtgggtttgatccctggcctcactcagtgggttaaggatccggtgttgccgtgagctgtggtgtaggttgcagacacggttctgatcctgcgttgctgtggctgtggctgtggtgtaggccagcagcaaacagctctgattagacccctagcctggaaacctccatatgccacaggtgcagccctaaaaagacaaaaaaagagaaaagacaaaaaaaaaaaaaaaaaaaaaaaaaaaaaaaaaaaaaaaaaaaagaacccccagaggtatttatttgtttttgccttttttcactgactgttctttgtttgtttgtttgagactgatctagaagactagagattacaagaaatatggatttggctcactctaagaaactgctttcattccaaggtttgggtctatccaaaagtggaatagaatcatatgaatactagtttatgagtatttagtgagaggaatttcaagctcaaataatgattcagcaagattaaattaaggagggaattttccttgtggctgagtgggttaaggacccaatgttgtctctgtgaggatgtaggttccatcctgggctttgctcattaggttaaggatctggcattgctgcagctcagacccagtgctgccctggttgtggcttaggccaaagctgcagctccaattcaatctctggcctgggaacctccatgtgctacaaggtgcggccttaaaaggaaaaaaaaaaaattaaatcaaggactcaagagtctttcattatttgtgttgtggaagctatatttgttttaaagtcttagttgtgtttagaaagcaagatgttcttcaactcaaatttgggagggaacttgtttcatacatttttaatggataagtggcaaaattttcatgctgaggtgatctatagtgttgtaatgcagaatatagtcagatcttgaacattttaggaagttggtgagggccaattgtgtatctgtgccatgctgataagaatgtcaagggatcacaagaattcgtgttatttgacagcagtcatctttaaaaggcatttgagaaagtccaatttcaaatgcatttcctttctttaaaagataaattgaagaaaataagtctttatttcccaagtaaattgaattgcctctcagtctgttaaaagaaactcttaccttgatgattgcgctcttaacctggcaaagattgtctttaaaatctgagctccatgtcttctgctttatttctggtgtgcctttgactccagattacagtaaatggaggactgagtatagggctaaaaagtagagagaatggatgcatattatctgtggtctccaatgtgatgaatgaagtaggcaaatactcaaaggaaagagaaagcatgctccaagaattatgggttccagaaggcaaagtcccagaattgtctccagggaaggacagggaggtctagaatcggctaagcccactgtaggcagaaaaaccaagaggcatgaatggcttccctttctcacttttcactctctggcttactcctatcatgaaggaaaatattggaatcatattctccctcaccgaaatgctatttttcagcccacaggaaacccagctcaacattcttgggtcctgggggtccctctgcaactctcactgggacatggaagatgcccatgttttatgccagcagcttaaatgtggagttgccctttctatcccgggaggagcaccttttgggaaaggaagtgagcaggtctggaggcacatgtttcactgcactgggactgagaagcacatgggagattgttccgtcactgctctgggcgcatcactctgttcttcagggcaagtggcctctgtaatctgctcaggtaagagaataagggcagccagtgatgagccactcatgacggtgccttaagagtgggtgtacctaggagttcccattgtggctcagtggtaacaaactcgactggtatccatgagggtatgggtttgatccctggccttgctcaatgggttaaggatccagcattgctgtgagctgtggtataggttgcagactctgctcaggtcccatgttgctgtgattgtggtgtaggctgactgctgcagcttcaatttgacccctagcccgggaatttccataggccacacgtgcagcactaaggaaggaaaaaaagaaaaaaaaaaaaaaagagtgggtgtgcctatagtgaagaacagatgtaaaagggaagtgaaagggattcccccattctgagggattgtgagaagtgtgccagaatattaacttcatttgacttgttacagggaaagtaaacttgactttcacggacctcctagttacctggtgcttactatatgtcttctcagagtacctgattcattcccagcctggttgacccatccccctatctctatggctatgtttatccagagcacatctatctaacactccagctgatcttcctgacacagctgtggcaaccctggatcctttaaccaactgtgccaggctggagatcaaacctaagcctctgcagcaacccaagctgctgcagtcagatttttaaccccctgtgccactgtgggtatctccgatattttgtatcttctgtgactgagtggtttgctgtttgcagggaaccagagtcagacactatccccgtgcaattcatcatcctcggacccatcaagctctattatttcagaagaaaatggtgttgcctgcataggtgagaatcagtgaccaacctatgaaaatgatctcaatcctctgaaatgcattttattcatgttttatttcctctttgcagggagtggtcaacttcgcctggtcgatggaggtggtcgttgtgctgggagagtagaggtctatcatgagggctcctggggcaccatctgtgatgacagctgggacctgaatgatgcccatgtggtgtgcaaacagctgagctgtggatgggccattaatgccactggttctgctcattttggggaaggaacagggcccatttggctggatgagataaactgtaatggaaaagaatctcatatttggcaatgccactcacatggttgggggcggcacaattgcaggcataaggaggatgcaggagtcatctgctcgg

SEQ ID NO: 120 - protein, 101 aa, Sus scrofa
PRLVGGDIPCSGRVEVQHGDTWGTVCDSDFSLEAASVLCRELQCGTVVSLLGGAHFGEGSGQIWAEEFQCEGHESHLSLCPVAPRPDGTCSHSRDVGVVCS

SEQ ID NO: 121 - protein, 100 aa, Homo sapiens
LRLVDGDSRCAGRVEIYHDGFWGTICDDGWDLSDAHVVCQKLGCGVAFNATVSAHFGEGSGPIWLDDLNCTGMESHLWQCPSRGWGQHDCRHKEDAGVIC